European Patent Application EP 4 431 609 A1, published September 18, 2024. Title: METHOD FOR IMPROVING 2, 4 DIHYDROXYBUTYRIC ACID PRODUCTION AND YIELD. Applicant: ADISSEO FRANCE S.A.S. The sequence listing filed with the application follows.

SEQUENCE LISTING (131 sequences)

SEQ ID NO: 1 - DNA, 909 bp, Escherichia coli
  source 1..909: mol_type = genomic DNA
atgccgcagtccgcgttgttcacgggaatcattccccctgtctccaccatttttaccgccgacggccagctcgataagccgggcaccgccgcgctgatcgacgatctgatcaaagcaggcgttgacggcctgttcttcctgggcagcggtggcgagttctcccagctcggcgccgaagagcgtaaagccattgcccgctttgctatcgatcatgtcgatcgtcgcgtgccggtgctgatcggcaccggcggcaccaacgcccgggaaaccatcgaactcagccagcacgcgcagcaggcgggcgcggacggcatcgtggtgatcaacccctactactggaaagtgtcggaagcgaacctgatccgctatttcgagcaggtggccgacagcgtcacgctgccggtgatgctctataacttcccggcgctgaccgggcaggatctgactccggcgctggtgaaaaccctcgccgactcgcgcagcaatattatcggcatcaaagacaccatcgactccgtcgcccacctgcgcagcatgatccataccgtcaaaggtgcccatccgcacttcaccgtgctctgcggctacgacgatcatctgttcaataccctgctgctcggcggcgacggggcgatatcggcgagcggcaactttgccccgcaggtgtcggtgaatcttctgaaagcctggcgcgacggggacgtggcgaaagcggccgggtatcatcagaccttgctgcaaattccgcagatgtatcagctggatacgccgtttgtgaacgtgattaaagaggcgatcgtgctctgcggtcgtcctgtctccacgcacgtgctgccgcccgcctcgccgctggacgagccgcgcaaggcgcagctgaaaaccctgctgcaacagctcaagctttgctga

SEQ ID NO: 2 - protein, 302 aa, Escherichia coli
MPQSALFTGIIPPVSTIFTADGQLDKPGTAALIDDLIKAGVDGLFFLGSGGEFSQLGAEERKAIARFAIDHVDRRVPVLIGTGGTNARETIELSQHAQQAGADGIVVINPYYWKVSEANLIRYFEQVADSVTLPVMLYNFPALTGQDLTPALVKTLADSRSNIIGIKDTIDSVAHLRSMIHTVKGAHPHFTVLCGYDDHLFNTLLLGGDGAISASGNFAPQVSVNLLKAWRDGDVAKAAGYHQTLLQIPQMYQLDTPFVNVIKEAIVLCGRPVSTHVLPPASPLDEPRKAQLKTLLQQLKLC

SEQ ID NO: 3 - DNA, 906 bp, Escherichia coli
  source 1..906: mol_type = genomic DNA
atgaaaaaattcagcggcattattccaccggtatccagcacgtttcatcgtgacggaacccttgataaaaaggcaatgcgcgaagttgccgacttcctgattaataaaggggtcgacgggctgttttatctgggtaccggtggtgaatttagccaaatgaatacagcccagcgcatggcactcgccgaagaagctgtaaccattgtcgacgggcgagtgccggtattgattggcgtcggttccccttccactgacgaagcggtcaaactggcgcagcatgcgcaagcctacggcgctgatggtatcgtcgccatcaacccctactactggaaagtcgcaccacgaaatcttgacgactattaccagcagatcgcccgtagcgtcaccctaccggtgatcctgtacaactttccggatctgacgggtcaggacttaaccccggaaaccgtgacgcgtctggctctgcaaaacgagaatatcgttggcatcaaagacaccatcgacagcgttggtcacttgcgtacgatgatcaacacagttaagtcggtacgcccgtcgttttcggtattctgcggttacgatgatcatttgctgaatacgatgctgctgggcggcgacggtgcgataaccgccagcgctaactttgctccggaactctccgtcggcatctaccgcgcctggcgtgaaggcgatctggcgaccgctgcgacgctgaataaaaaactactacaactgcccgctatttacgccctcgaaacaccgtttgtctcactgatcaaatacagcatgcagtgtgtcgggctgcctgtagagacatattgcttaccaccgattcttgaagcatctgaagaagcaaaagataaagtccacgtgctgcttaccgcgcagggcattttaccagtctga

SEQ ID NO: 4 - protein, 301 aa, Escherichia coli
MKKFSGIIPPVSSTFHRDGTLDKKAMREVADFLINKGVDGLFYLGTGGEFSQMNTAQRMALAEEAVTIVDGRVPVLIGVGSPSTDEAVKLAQHAQAYGADGIVAINPYYWKVAPRNLDDYYQQIARSVTLPVILYNFPDLTGQDLTPETVTRLALQNENIVGIKDTIDSVGHLRTMINTVKSVRPSFSVFCGYDDHLLNTMLLGGDGAITASANFAPELSVGIYRAWREGDLATAATLNKKLLQLPAIYALETPFVSLIKYSMQCVGLPVETYCLPPILEASEEAKDKVHVLLTAQGILPV

SEQ ID NO: 5 - DNA, 930 bp, Escherichia coli
  source 1..930: mol_type = genomic DNA
atgaccacgaagaaagctgattacatttggttcaatggggagatggttcgctgggaagacgcgaaggtgcatgtgatgtcgcacgcgctgcactatggcacttcggtttttgaaggcatccgttgctacgactcgcacaaaggaccggttgtattccgccatcgtgagcatatgcagcgtctgcatgactccgccaaaatctatcgcttcccggtttcgcagagcattgatgagctgatggaagcttgtcgtgacgtgatccgcaaaaacaatctcaccagcgcctatatccgtccgctgatcttcgtcggtgatgttggcatgggagtaaacccgccagcgggatactcaaccgacgtgattatcgctgctttcccgtggggagcgtatctgggcgcagaagcgctggagcaggggatcgatgcgatggtttcctcctggaaccgcgcagcaccaaacaccatcccgacggcggcaaaagccggtggtaactacctctcttccctgctggtgggtagcgaagcgcgccgccacggttatcaggaaggtatcgcgctggatgtgaacggttatatctctgaaggcgcaggcgaaaacctgtttgaagtgaaagatggtgtgctgttcaccccaccgttcacctcctccgcgctgccgggtattacccgtgatgccatcatcaaactggcgaaagagctgggaattgaagtacgtgagcaggtgctgtcgcgcgaatccctgtacctggcggatgaagtgtttatgtccggtacggcggcagaaatcacgccagtgcgcagcgtagacggtattcaggttggcgaaggccgttgtggcccggttaccaaacgcattcagcaagccttcttcggcctcttcactggcgaaaccgaagataaatggggctggttagatcaagttaatcaataa

SEQ ID NO: 6 - protein, 309 aa, Escherichia coli
MTTKKADYIWFNGEMVRWEDAKVHVMSHALHYGTSVFEGIRCYDSHKGPVVFRHREHMQRLHDSAKIYRFPVSQSIDELMEACRDVIRKNNLTSAYIRPLIFVGDVGMGVNPPAGYSTDVIIAAFPWGAYLGAEALEQGIDAMVSSWNRAAPNTIPTAAKAGGNYLSSLLVGSEARRHGYQEGIALDVNGYISEGAGENLFEVKDGVLFTPPFTSSALPGITRDAIIKLAKELGIEVREQVLSRESLYLADEVFMSGTAAEITPVRSVDGIQVGEGRCGPVTKRIQQAFFGLFTGETEDKWGWLDQVNQ

SEQ ID NO: 7 - DNA, 1194 bp, Escherichia coli
  source 1..1194: mol_type = genomic DNA
gtgtttcaaaaagttgacgcctacgctggcgacccgattcttacgcttatggagcgttttaaagaagaccctcgcagcgacaaagtgaatttaagtatcggtctgtactacaacgaagacggaattattccacaactgcaagccgtggcggaggcggaagcgcgcctgaatgcgcagcctcatggcgcttcgctttatttaccgatggaagggcttaactgctatcgccatgccattgcgccgctgctgtttggtgcggaccatccggtactgaaacaacagcgcgtagcaaccattcaaacccttggcggctccggggcattgaaagtgggcgcggatttcctgaaacgctacttcccggaatcaggcgtctgggtcagcgatcctacctgggaaaaccacgtagcaatattcgccggggctggattcgaagtgagtacttacccctggtatgacgaagcgactaacggcgtgcgctttaatgacctgttggcgacgctgaaaacattacctgcccgcagtattgtgttgctgcatccatgttgccacaacccaacgggtgccgatctcactaatgatcagtgggatgcggtgattgaaattctcaaagcccgcgagcttattccattcctcgatattgcctatcaaggatttggtgccggtatggaagaggatgcctacgctattcgcgccattgccagcgctggattacccgctctggtgagcaattcgttctcgaaaattttctccctttacggcgagcgcgtcggcggactttctgttatgtgtgaagatgccgaagccgctggccgcgtactggggcaattgaaagcaacagttcgccgcaactactccagcccgccgaattttggtgcgcaggtggtggctgcagtgctgaatgacgaggcattgaaagccagctggctggcggaagtagaagagatgcgtactcgcattctggcaatgcgtcaggaattggtgaaggtattaagcacagagatgccagaacgcaatttcgattatctgcttaatcagcgcggcatgttcagttataccggtttaagtgccgctcaggttgaccgactacgtgaagaatttggtgtctatctcatcgccagcggtcgcatgtgtgtcgccgggttaaatacggcaaatgtacaacgtgtggcaaaggcgtttgctgcggtgatgtaa

SEQ ID NO: 8 - protein, 397 aa, Escherichia coli
VFQKVDAYAGDPILTLMERFKEDPRSDKVNLSIGLYYNEDGIIPQLQAVAEAEARLNAQPHGASLYLPMEGLNCYRHAIAPLLFGADHPVLKQQRVATIQTLGGSGALKVGADFLKRYFPESGVWVSDPTWENHVAIFAGAGFEVSTYPWYDEATNGVRFNDLLATLKTLPARSIVLLHPCCHNPTGADLTNDQWDAVIEILKARELIPFLDIAYQGFGAGMEEDAYAIRAIASAGLPALVSNSFSKIFSLYGERVGGLSVMCEDAEAAGRVLGQLKATVRRNYSSPPNFGAQVVAAVLNDEALKASWLAEVEEMRTRILAMRQELVKVLSTEMPERNFDYLLNQRGMFSYTGLSAAQVDRLREEFGVYLIASGRMCVAGLNTANVQRVAKAFAAVM

SEQ ID NO: 9 - DNA, 1191 bp, Escherichia coli
  source 1..1191: mol_type = genomic DNA
atgtttgagaacattaccgccgctcctgccgacccgattctgggcctggccgatctgtttcgtgccgatgaacgtcccggcaaaattaacctcgggattggtgtctataaagatgagacgggcaaaaccccggtactgaccagcgtgaaaaaggctgaacagtatctgctcgaaaatgaaaccaccaaaaattacctcggcattgacggcatccctgaatttggtcgctgcactcaggaactgctgtttggtaaaggtagcgccctgatcaatgacaaacgtgctcgcacggcacagactccggggggcactggcgcactacgcgtggctgccgatttcctggcaaaaaataccagcgttaagcgtgtgtgggtgagcaacccaagctggccgaaccataagagcgtctttaactctgcaggtctggaagttcgtgaatacgcttattatgatgcggaaaatcacactcttgacttcgatgcactgattaacagcctgaatgaagctcaggctggcgacgtagtgctgttccatggctgctgccataacccaaccggtatcgaccctacgctggaacaatggcaaacactggcacaactctccgttgagaaaggctggttaccgctgtttgacttcgcttaccagggttttgcccgtggtctggaagaagatgctgaaggactgcgcgctttcgcggctatgcataaagagctgattgttgccagttcctactctaaaaactttggcctgtacaacgagcgtgttggcgcttgtactctggttgctgccgacagtgaaaccgttgatcgcgcattcagccaaatgaaagcggcgattcgcgctaactactctaacccaccagcacacggcgcttctgttgttgccaccatcctgagcaacgatgcgttacgtgcgatttgggaacaagagctgactgatatgcgccagcgtattcagcgtatgcgtcagttgttcgtcaatacgctgcaggaaaaaggcgcaaaccgcgacttcagctttatcatcaaacagaacggcatgttctccttcagtggcctgacaaaagaacaagtgctgcgtctgcgcgaagagtttggcgtatatgcggttgcttctggtcgcgtaaatgtggccgggatgacaccagataacatggctccgctgtgcgaagcgattgtggcagtgctgtaa

SEQ ID NO: 10 - protein, 396 aa, Escherichia coli
MFENITAAPADPILGLADLFRADERPGKINLGIGVYKDETGKTPVLTSVKKAEQYLLENETTKNYLGIDGIPEFGRCTQELLFGKGSALINDKRARTAQTPGGTGALRVAADFLAKNTSVKRVWVSNPSWPNHKSVFNSAGLEVREYAYYDAENHTLDFDALINSLNEAQAGDVVLFHGCCHNPTGIDPTLEQWQTLAQLSVEKGWLPLFDFAYQGFARGLEEDAEGLRAFAAMHKELIVASSYSKNFGLYNERVGACTLVAADSETVDRAFSQMKAAIRANYSNPPAHGASVVATILSNDALRAIWEQELTDMRQRIQRMRQLFVNTLQEKGANRDFSFIIKQNGMFSFSGLTKEQVLRLREEFGVYAVASGRVNVAGMTPDNMAPLCEAIVAVL

SEQ ID NO: 11 - DNA, 1176 bp, Lactobacillus lactis
  source 1..1176: mol_type = genomic DNA
atggatttattaaaaaaatttaaccctaatttagataaaattgaaatttcattgattcgtcagtttgaccaacaggtttcatctattcctgatgttattaagttgactttgggagaacctgatttttatacgcctgagcatgttaaacaagcagggattgtggcgattgaaaataatcaaagtcattatactggaatggctggtttactagaactacgtcaggcagctagtgaatttatgaataaaaaatatggtttatcttatgcagcagaagatgaaattttagttactgttggagtaacggaagccatttctagtgttttgttatcaattttggttgctggtgatgaagttttgattcccgcgcctgcatatcctggttatgagccattaattacgcttgctggcggttctttggttgaaattgatacaagagctaatgattttgttcttacgcctgagatgcttgaacaagcgattgtcgagcgtgagggaaaagttaaggccgttattttgaattatccagcaaatcctacaggggtaacttataatcgggggcaaattaaggctttagctgaagttttgaaaaagcatgaagtatttgtgattgctgatgaagtttattctgaactaaattatactgaccaaccgcatgtgtcaattgctgaatatgcacctgagcaaacaatcgttcttaatggtttatcaaaatcgcatgcgatgactggttggcggattggattaatctttgcagcgcgtgaattagtggcacagattattaagactcaccaatatttggtgacttcggcttcaactcagtcacagtttgcagcgattgaagctttgaaaaatggtgcttatgatgctcttccgatgaaaaaagaatatcttaaacgtcgtgattatattattgaaaagatgtcagaccttggtttcaaaattattgaaccagatggagctttctacatttttgcaaaaattccagctgatttagaacaagattcattcaaatttgctgtggattttgcaaaagaaaatgcagttgccattattcctggtatcgcttttggtcagtacggtgaaggatttgtccgcttatcttatgcggcttcaatggatatgattgagcaagcaatggcaagattgacggattatgtgactaaaaaacgtggctga

SEQ ID NO: 12 - protein, 391 aa, Lactobacillus lactis
MDLLKKFNPNLDKIEISLIRQFDQQVSSIPDVIKLTLGEPDFYTPEHVKQAGIVAIENNQSHYTGMAGLLELRQAASEFMNKKYGLSYAAEDEILVTVGVTEAISSVLLSILVAGDEVLIPAPAYPGYEPLITLAGGSLVEIDTRANDFVLTPEMLEQAIVEREGKVKAVILNYPANPTGVTYNRGQIKALAEVLKKHEVFVIADEVYSELNYTDQPHVSIAEYAPEQTIVLNGLSKSHAMTGWRIGLIFAARELVAQIIKTHQYLVTSASTQSQFAAIEALKNGAYDALPMKKEYLKRRDYIIEKMSDLGFKIIEPDGAFYIFAKIPADLEQDSFKFAVDFAKENAVAIIPGIAFGQYGEGFVRLSYAASMDMIEQAMARLTDYVTKKRG

SEQ ID NO: 13 - DNA, 1023 bp, Lactococcus lactis
  source 1..1023: mol_type = genomic DNA
atggcaattaatttagactgggaaaatttaggattcagctatcggaacttaccttttcgttatatcgctcgttttaaagatggaaaatggagtgctggagaactaacaggagataatcaacttcatattagtgaatcatcacctgctttgcattatggtcaacaaggttttgaaggattaaaagcctatcgaacaaaggatggttcaatccaacttttccgtcctgaccaaaatgctgctcgtttgcaaaatacggcgcgtcgactttgcatggcagaagttccaactgaaatgtttattgatgcagttaaacaagtggtgaaagcaaacgaagattttgtgcctccttacggaacgggtgcaacgctctatctccgtccacttttgattggggttggtgacgttattggggtgaaacctgctgatgaatatattttcaccgtttttgctatgccggttggttcttattttaaaggcggattggctccttcaaaatttgtaatttcaagagattatgatagggcagctccacttggtacaggtggtgccaaagttggaggaaattatgcagcttctttacaagcagaagttggtgccaaagcttcaggctatgcagatgcaatttatcttgacccaagcacacatactaaaattgaagaagtcggggcagcaaatttctttggaattacagccgataatgaatttatcacaccattgagtccatcaatcttaccttcaattactaaatattctcttctttatttagctgaacatcgtttgggactcaaagcgattgagggtgaagtttatgccaaagatttaggtaaatttgttgaagcaggagcttgtggcacagcggcaattatctctccaattggtcgtattgacgatggagaagattcttacattttccattcagaaacagaagtaggaccaacggttaaacgtttatatgatgagttggttggcattcagtttggtgatgttgaagcaccagaaggctggatagttaaagttgattaa

SEQ ID NO: 14 - protein, 340 aa, Lactococcus lactis
MAINLDWENLGFSYRNLPFRYIARFKDGKWSAGELTGDNQLHISESSPALHYGQQGFEGLKAYRTKDGSIQLFRPDQNAARLQNTARRLCMAEVPTEMFIDAVKQVVKANEDFVPPYGTGATLYLRPLLIGVGDVIGVKPADEYIFTVFAMPVGSYFKGGLAPSKFVISRDYDRAAPLGTGGAKVGGNYAASLQAEVGAKASGYADAIYLDPSTHTKIEEVGAANFFGITADNEFITPLSPSILPSITKYSLLYLAEHRLGLKAIEGEVYAKDLGKFVEAGACGTAAIISPIGRIDDGEDSYIFHSETEVGPTVKRLYDELVGIQFGDVEAPEGWIVKVD

SEQ ID NO: 15 - DNA, 1503 bp, Saccharomyces cerevisiae
  source 1..1503: mol_type = genomic DNA
atgactttacctgaatcaaaagacttttcttacttgttttcggatgaaaccaatgctcgtaaaccatccccattgaaaacctgcatccatcttttccaagatcctaacattatctttttgggtggtggcctgccattaaaagattatttcccatgggataatctatctgtagattcacccaagcctccttttccccagggtattggagctccaattgacgagcagaattgcataaaatacaccgtcaacaaagattacgctgataaaagtgccaatccttccaacgatattcctttgtcaagagctttgcaatacgggttcagtgctggtcaacctgaactattaaacttcattagagatcataccaagattatccacgatttgaagtataaggactgggacgttttagccactgcaggtaacacaaatgcctgggaatctactttaagagtcttttgtaaccgaggtgatgtcatcttagttgaggcacattctttttcctcttcattggcttctgcagaggctcaaggtgtcattaccttccccgtgccaattgacgctgatggtatcattcctgaaaaattagctaaagtcatggaaaactggacacctggtgctcctaaaccaaagttgttatacactattccaacgggccaaaatccaactggtacttccattgcagaccatagaaaggaggcaatttacaagatcgctcaaaagtacgacttcctaattgtggaagatgaaccttattatttcttacaaatgaatccctacatcaaagacttgaaggaaagagagaaggcacaaagttctccaaagcaggaccatgacgaatttttgaagtccttggcaaacactttcctttccttggatacagaaggccgtgttattagaatggattccttttcaaaagttttggccccagggacaagattgggttggattactggttcatccaaaatcttgaagccttacttgagtttgcatgaaatgacgattcaagccccagcaggttttacacaagttttggtcaacgctacgctatccaggtggggtcaaaagggttacttggactggttgcttggcctgcgtcatgaatacactttgaaacgtgactgtgccatcgatgccctttacaagtatctaccacaatctgatgctttcgtgatcaatcctccaattgcaggtatgtttttcaccgtgaacattgacgcatctgtccaccctgagtttaaaacaaaatacaactcagacccttaccagctagaacagagtctttaccacaaagtggttgaacgtggtgttttagtggttcccggttcttggttcaagagtgagggtgagacggaacctcctcaacccgctgaatctaaagaagtcagtaatccaaacataattttcttcagaggtacctatgcagctgtctctcctgagaaactgactgaaggtctgaagagattaggtgatactttatacgaagaatttggtatttccaaatag

SEQ ID NO: 16 - protein, 500 aa, Saccharomyces cerevisiae
MTLPESKDFSYLFSDETNARKPSPLKTCIHLFQDPNIIFLGGGLPLKDYFPWDNLSVDSPKPPFPQGIGAPIDEQNCIKYTVNKDYADKSANPSNDIPLSRALQYGFSAGQPELLNFIRDHTKIIHDLKYKDWDVLATAGNTNAWESTLRVFCNRGDVILVEAHSFSSSLASAEAQGVITFPVPIDADGIIPEKLAKVMENWTPGAPKPKLLYTIPTGQNPTGTSIADHRKEAIYKIAQKYDFLIVEDEPYYFLQMNPYIKDLKEREKAQSSPKQDHDEFLKSLANTFLSLDTEGRVIRMDSFSKVLAPGTRLGWITGSSKILKPYLSLHEMTIQAPAGFTQVLVNATLSRWGQKGYLDWLLGLRHEYTLKRDCAIDALYKYLPQSDAFVINPPIAGMFFTVNIDASVHPEFKTKYNSDPYQLEQSLYHKVVERGVLVVPGSWFKSEGETEPPQPAESKEVSNPNIIFFRGTYAAVSPEKLTEGLKRLGDTLYEEFGISK

SEQ ID NO: 17 - DNA, 978 bp, Lactococcus lactis
  source 1..978: mol_type = genomic DNA
atggctgataaacaacgtaaaaaagttatccttgtaggtgacggtgctgtaggttcatcatacgcttttgctcttgtaaaccaagggattgcacaagaattaggaattgttgacctttttaaagaaaaaactcaaggagatgcagaagacctttctcatgccttggcatttacttcacctaaaaagatttactctgcagactattctgatgcaagcgacgctgacctcgttgtcttgacttctggtgctccacaaaaaccaggtgaaactcgtcttgaccttgttgaaaaaaatcttcgtatcactaaagatgttgtcactaaaattgttgcttcaggtttcaaaggaatcttccttgttgctgctaacccagttgatatcttgacatacgctacttggaaattctcaggtttccctaaaaaccgcgttgtaggttcaggtacttcacttgatactgcacgtttccgtcaagcattggcagaaaaagttgatgttgacgctcgttcaatccacgcatacatcatgggtgaacacggtgactcagaatttgccgtttggtcacacgctaacgttgctggtgttaaattggaacaatggttccaagaaaatgactaccttaacgaagctgaaatcgttgaattgtttgaatctgtacgtgatgctgcttactcaatcatcgctaaaaaaggtgcaacattctatggtgtcgctgtagctcttgctcgtattactaaagcaattcttgatgatgaacatgcagtacttccagtatcagtatttcaagatggacaatatggcgtaagcgactgctaccttggtcaaccagctgtagttggtgctgaaggtgttgttaacccaatccacattccattgaatgatgctgaaatgcaaaaaatggaagcttctggtgctcaattgaaagcaatcattgacgaagcttttgctaaagaagaatttgcttctgcagttaaaaactaa

SEQ ID NO: 18 - protein, 325 aa, Lactococcus lactis
MADKQRKKVILVGDGAVGSSYAFALVNQGIAQELGIVDLFKEKTQGDAEDLSHALAFTSPKKIYSADYSDASDADLVVLTSGAPQKPGETRLDLVEKNLRITKDVVTKIVASGFKGIFLVAANPVDILTYATWKFSGFPKNRVVGSGTSLDTARLRQALAEKVDVDARSIHAYIMGEHGDSEFAVWSHANVAGVKLEQWFQENDYLNEAEIVELFESVRDAAYSIIAKKGATFYGVAVALARITKAILDDEHAVLPVSVFQDGQYGVSDCYLGQPAVVGAEGVVNPIHIPLNDAEMQKMEASGAQLKAIIDEAFAKEEFASAVKN

SEQ ID NO: 19 - DNA, 939 bp, Escherichia coli
  source 1..939: mol_type = genomic DNA
atgaaagtcgcagtcctcggcgctgctggcggtattggccaggcgcttgcactactgttaaaaacccaactgccttcaggttcagaactctctctgtatgatatcgctccagtgactcccggtgtggctgtcgatctgagccatatccctactgctgtgaaaatcaaaggtttttctggtgaagatgcgactccggcgctggaaggcgcagatgtcgttcttatctctgcaggcgtagcgcgtaaaccgggtatggatcgttccgacctgtttaacgttaacgccggcatcgtgaaaaacctggtacagcaagttgcgaaaacctgcccgaaagcgtgcattggtattatcactaacccggttaacaccacagttgcaattgctgctgaagtgctgaaaaaagccggtgtttatgacaaaaacaaactgttcggcgttaccacgctggatatcattcgttccaacacctttgttgcggaactgaaaggcaaacagccaggcgaagttgaagtgccggttattggcggtcactctggtgttaccattctgccgctgctgtcacaggttcctggcgttagttttaccgagcaggaagtggctgatctgaccaaacgcatccagaacgcgggtactgaagtggttgaagcgaaggccggtggcgggtctgcaaccctgtctatgggccaggcagctgcacgttttggtctgtctctggttcgtgcactgcagggcgaacaaggcgttgtcgaatgtgcctacgttgaaggcgacggtcagtacgcccgtttcttctctcaaccgctgctgctgggtaaaaacggcgtggaagagcgtaaatctatcggtaccctgagcgcatttgaacagaacgcgctggaaggtatgctggatacgctgaagaaagatatcgccctgggcgaagagttcgttaataagtaa

SEQ ID NO: 20 - protein, 312 aa, Escherichia coli
MKVAVLGAAGGIGQALALLLKTQLPSGSELSLYDIAPVTPGVAVDLSHIPTAVKIKGFSGEDATPALEGADVVLISAGVARKPGMDRSDLFNVNAGIVKNLVQQVAKTCPKACIGIITNPVNTTVAIAAEVLKKAGVYDKNKLFGVTTLDIIRSNTFVAELKGKQPGEVEVPVIGGHSGVTILPLLSQVPGVSFTEQEVADLTKRIQNAGTEVVEAKAGGGSATLSMGQAAARFGLSLVRALQGEQGVVECAYVEGDGQYARFFSQPLLLGKNGVEERKSIGTLSAFEQNALEGMLDTLKKDIALGEEFVNK

SEQ ID NO: 21 - DNA, 978 bp, Lactococcus lactis
  source 1..978: mol_type = genomic DNA
atggctgataaacaacgtaaaaaagttatccttgtaggtgacggtgctgtaggttcatcatacgcttttgctcttgtaaaccaagggattgcacaagaattaggaattgttgacctttttaaagaaaaaactcaaggagatgcagaagacctttctcatgccttggcatttacttcacctaaaaagatttactctgcagactattctgatgcaagcgacgctgacctcgttgtcttgacttctggtgctccaaacaaaccaggtgaaactcgtcttgaccttgttgaaaaaaatcttcgtatcactaaagatgttgtcactaaaattgttgcttcaggtttcaaaggaatcttccttgttgctgctaacccagttgatatcttgacatacgctacttggaaattctcaggtttccctaaaaaccgcgttgtaggttcaggtacttcacttgatactgcacgtttccgtcaagcattggcagaaaaagttgatgttgacgctcgttcaatccacgcatacatcatgggtgaacacggtgactcagaatttgccgtttggtcacacgctaacgttgctggtgttaaattggaacaatggttccaagaaaatgactaccttaacgaagctgaaatcgttgaattgtttgaatctgtacgtgatgctgcttactcaatcatcgctaaaaaaggtgcaacattctatggtgtcgctgtagctcttgctcgtattactaaagcaattcttgatgatgaacatgcagtacttccagtatcagtatttcaagatggacaatatggcgtaagcgactgctaccttggtcaaccagctgtagttggtgctgaaggtgttgttaacccaatccacattccattgaatgatgctgaaatgcaaaaaatggaagcttctggtgctcaattgaaagcaatcattgacgaagcttttgctaaagaagaatttgcttctgcagttaaaaactaa

SEQ ID NO: 22 - protein, 325 aa, Lactococcus lactis
MADKQRKKVILVGDGAVGSSYAFALVNQGIAQELGIVDLFKEKTQGDAEDLSHALAFTSPKKIYSADYSDASDADLVVLTSGAPNKPGETRLDLVEKNLRITKDVVTKIVASGFKGIFLVAANPVDILTYATWKFSGFPKNRVVGSGTSLDTARLRQALAEKVDVDARSIHAYIMGEHGDSEFAVWSHANVAGVKLEQWFQENDYLNEAEIVELFESVRDAAYSIIAKKGATFYGVAVALARITKAILDDEHAVLPVSVFQDGQYGVSDCYLGQPAVVGAEGVVNPIHIPLNDAEMQKMEASGAQLKAIIDEAFAKEEFASAVKN

SEQ ID NO: 23 - DNA, 978 bp, Lactococcus lactis
  source 1..978: mol_type = genomic DNA
atggctgataaacaacgtaaaaaagttatccttgtaggtgacggtgctgtaggttcatcatacgcttttgctcttgtaaaccaagggattgcacaagaattaggaattgttgacctttttaaagaaaaaactcaaggagatgcagaagacctttctcatgccttggcatttacttcacctaaaaagatttactctgcagactattctgatgcaagcgacgctgacctcgttgtcttgacttctggtgctccacaaaaaccaggtgaaactcgtcttgaccttgttgaaaaaaatcttcgtatcactaaagatgttgtcactaaaattgttgcttcaggtttcaaaggaatcttccttgttgctgctaacccagttgatatcttgacatacgctacttggaaattctcaggtttccctaaaaaccgcgttgtaggttcaggtacttcacttgatactgcacgtttccgtcaagcattggcagaaaaagttgatgttgacgctcgttcaatccacgcatacatcatgggtgaacacggtgactcagaatttgccgtttggtcacacgctaacgttgctggtgttaaattggaacaatggttccaagaaaatgactaccttaacgaagctgaaatcgttgaattgtttgaatctgtacgtgatgctgcttactcaatcgtcgctaaaaaaggtgcaacattctatggtgtcgctgtagctcttgctcgtattactaaagcaattcttgatgatgaacatgcagtacttccagtatcagtatttcaagatggacaatatggcgtaagcgactgctaccttggtcaaccagctgtagttggtgctgaaggtgttgttaacccaatccacattccattgaatgatgctgaaatgcaaaaaatggaagcttctggtgctcaattgaaagcaatcattgacgaagcttttgctaaagaagaatttgcttctgcagttaaaaactaa

SEQ ID NO: 24 - protein, 325 aa, Lactococcus lactis
MADKQRKKVILVGDGAVGSSYAFALVNQGIAQELGIVDLFKEKTQGDAEDLSHALAFTSPKKIYSADYSDASDADLVVLTSGAPQKPGETRLDLVEKNLRITKDVVTKIVASGFKGIFLVAANPVDILTYATWKFSGFPKNRVVGSGTSLDTARLRQALAEKVDVDARSIHAYIMGEHGDSEFAVWSHANVAGVKLEQWFQENDYLNEAEIVELFESVRDAAYSIVAKKGATFYGVAVALARITKAILDDEHAVLPVSVFQDGQYGVSDCYLGQPAVVGAEGVVNPIHIPLNDAEMQKMEASGAQLKAIIDEAFAKEEFASAVKN

SEQ ID NO: 25 - DNA, 978 bp, Lactococcus lactis
  source 1..978: mol_type = genomic DNA
atggctgataaacaacgtaaaaaagttatccttgtaggtgacggtgctgtaggttcatcatacgcttttgctcttgtaaaccaagggattgcacaagaattaggaattgttgacctttttaaagaaaaaactcaaggagatgcagaagacctttctcatgccttggcatttacttcacctaaaaagatttactctgcagactattctgatgcaagcgacgctgacctcgttgtcttgacttctggtgctccaaacaaaccaggtgaaactcgtcttgaccttgttgaaaaaaatcttcgtatcactaaagatgttgtcactaaaattgttgcttcaggtttcaaaggaatcttccttgttgctgctaacccagttgatatcttgacatacgctacttggaaattctcaggtttccctaaaaaccgcgttgtaggttcaggtacttcacttgatactgcacgtttccgtcaagcattggcagaaaaagttgatgttgacgctcgttcaatccacgcatacatcatgggtgaacacggtgactcagaatttgccgtttggtcacacgctaacgttgctggtgttaaattggaacaatggttccaagaaaatgactaccttaacgaagctgaaatcgttgaattgtttgaatctgtacgtgatgctgcttactcaatcgtcgctaaaaaaggtgcaacattctatggtgtcgctgtagctcttgctcgtattactaaagcaattcttgatgatgaacatgcagtacttccagtatcagtatttcaagatggacaatatggcgtaagcgactgctaccttggtcaaccagctgtagttggtgctgaaggtgttgttaacccaatccacattccattgaatgatgctgaaatgcaaaaaatggaagcttctggtgctcaattgaaagcaatcattgacgaagcttttgctaaagaagaatttgcttctgcagttaaaaactaa

SEQ ID NO: 26 - protein, 325 aa, Lactococcus lactis
MADKQRKKVILVGDGAVGSSYAFALVNQGIAQELGIVDLFKEKTQGDAEDLSHALAFTSPKKIYSADYSDASDADLVVLTSGAPNKPGETRLDLVEKNLRITKDVVTKIVASGFKGIFLVAANPVDILTYATWKFSGFPKNRVVGSGTSLDTARLRQALAEKVDVDARSIHAYIMGEHGDSEFAVWSHANVAGVKLEQWFQENDYLNEAEIVELFESVRDAAYSIVAKKGATFYGVAVALARITKAILDDEHAVLPVSVFQDGQYGVSDCYLGQPAVVGAEGVVNPIHIPLNDAEMQKMEASGAQLKAIIDEAFAKEEFASAVKN

SEQ ID NO: 27 - DNA, 939 bp, Escherichia coli
  source 1..939: mol_type = genomic DNA
atgaaagtcgcagtcctcggcgctgctggcggtattggccaggcgcttgcactactgttaaaaacccaactgccttcaggttcagaactctctctgtatgatatcgctccagtgactcccggtgtggctgtcgatctgagccatatccctactgctgtgaaaatcaaaggtttttctggtgaagatgcgactccggcgctggaaggcgcagatgtcgttcttatctctgcaggcgtagcggctaaaccgggtatggatcgttccgacctgtttaacgttaacgccggcatcgtgaaaaacctggtacagcaagttgcgaaaacctgcccgaaagcgtgcattggtattatcactaacccggttaacaccacagttgcaattgctgctgaagtgctgaaaaaagccggtgtttatgacaaaaacaaactgttcggcgttaccacgctggatatcattcgttccaacacctttgttgcggaactgaaaggcaaacagccaggcgaagttgaagtgccggttattggcggtcactctggtgttaccattctgccgctgctgtcacaggttcctggcgttagttttaccgagcaggaagtggctgatctgaccaaacgcatccagaacgcgggtactgaagtggttgaagcgaaggccggtggcgggtctgcaaccctgtctatgggccaggcagctgcacgttttggtctgtctctggttcgtgcactgcagggcgaacaaggcgttgtcgaatgtgcctacgttgaaggcgacggtcagtacgcccgtttcttctctcaaccgctgctgctgggtaaaaacggcgtggaagagcgtaaatctatcggtaccctgagcgcatttgaacagaacgcgctggaaggtatgctggatacgctgaagaaagatatcgccctgggcgaagagttcgttaataagtaa

SEQ ID NO: 28 - protein, 312 aa, Escherichia coli
MKVAVLGAAGGIGQALALLLKTQLPSGSELSLYDIAPVTPGVAVDLSHIPTAVKIKGFSGEDATPALEGADVVLISAGVAAKPGMDRSDLFNVNAGIVKNLVQQVAKTCPKACIGIITNPVNTTVAIAAEVLKKAGVYDKNKLFGVTTLDIIRSNTFVAELKGKQPGEVEVPVIGGHSGVTILPLLSQVPGVSFTEQEVADLTKRIQNAGTEVVEAKAGGGSATLSMGQAAARFGLSLVRALQGEQGVVECAYVEGDGQYARFFSQPLLLGKNGVEERKSIGTLSAFEQNALEGMLDTLKKDIALGEEFVNK

SEQ ID NO: 29 - DNA, 939 bp, Escherichia coli
  source 1..939: mol_type = genomic DNA
atgaaagtcgcagtcctcggcgctgctggcggtattggccaggcgcttgcactactgttaaaaacccaactgccttcaggttcagaactctctctgtatgatatcgctccagtgactcccggtgtggctgtcgatctgagccatatccctactgctgtgaaaatcaaaggtttttctggtgaagatgcgactccggcgctggaaggcgcagatgtcgttcttatctctgcaggcgtagcggctaaaccgggtcaggatcgttccgacctgtttaacgttaacgccggcatcgtgaaaaacctggtacagcaagttgcgaaaacctgcccgaaagcgtgcattggtattatcactaacccggttaacaccacagttgcaattgctgctgaagtgctgaaaaaagccggtgtttatgacaaaaacaaactgttcggcgttaccacgctggatatcattcgttccaacacctttgttgcggaactgaaaggcaaacagccaggcgaagttgaagtgccggttattggcggtcactctggtgttaccattctgccgctgctgtcacaggttcctggcgttagttttaccgagcaggaagtggctgatctgaccaaacgcatccagaacgcgggtactgaagtggttgaagcgaaggccggtggcgggtctgcaaccctgtctatgggccaggcagctgcacgttttggtctgtctctggttcgtgcactgcagggcgaacaaggcgttgtcgaatgtgcctacgttgaaggcgacggtcagtacgcccgtttcttctctcaaccgctgctgctgggtaaaaacggcgtggaagagcgtaaatctatcggtaccctgagcgcatttgaacagaacgcgctggaaggtatgctggatacgctgaagaaagatatcgccctgggcgaagagttcgttaataagtaa

SEQ ID NO: 30 - protein, 312 aa, Escherichia coli
MKVAVLGAAGGIGQALALLLKTQLPSGSELSLYDIAPVTPGVAVDLSHIPTAVKIKGFSGEDATPALEGADVVLISAGVAAKPGQDRSDLFNVNAGIVKNLVQQVAKTCPKACIGIITNPVNTTVAIAAEVLKKAGVYDKNKLFGVTTLDIIRSNTFVAELKGKQPGEVEVPVIGGHSGVTILPLLSQVPGVSFTEQEVADLTKRIQNAGTEVVEAKAGGGSATLSMGQAAARFGLSLVRALQGEQGVVECAYVEGDGQYARFFSQPLLLGKNGVEERKSIGTLSAFEQNALEGMLDTLKKDIALGEEFVNK

SEQ ID NO: 31 - DNA, 939 bp, Escherichia coli
  source 1..939: mol_type = genomic DNA
atgaaagtcgcagtcctcggcgctgctggcggtattggccaggcgcttgcactactgttaaaaacccaactgccttcaggttcagaactctctctgtatgatatcgctccagtgactcccggtgtggctgtcgatctgagccatatccctactgctgtgaaaatcaaaggtttttctggtgaagatgcgactccggcgctggaaggcgcagatgtcgttcttatctctgcaggcgtagcggctaaaccgggtgaggatcgttccgacctgtttaacgttaacgccggcatcgtgaaaaacctggtacagcaagttgcgaaaacctgcccgaaagcgtgcattggtattatcactaacccggttaacaccacagttgcaattgctgctgaagtgctgaaaaaagccggtgtttatgacaaaaacaaactgttcggcgttaccacgctggatatcattcgttccaacacctttgttgcggaactgaaaggcaaacagccaggcgaagttgaagtgccggttattggcggtcactctggtgttaccattctgccgctgctgtcacaggttcctggcgttagttttaccgagcaggaagtggctgatctgaccaaacgcatccagaacgcgggtactgaagtggttgaagcgaaggccggtggcgggtctgcaaccctgtctatgggccaggcagctgcacgttttggtctgtctctggttcgtgcactgcagggcgaacaaggcgttgtcgaatgtgcctacgttgaaggcgacggtcagtacgcccgtttcttctctcaaccgctgctgctgggtaaaaacggcgtggaagagcgtaaatctatcggtaccctgagcgcatttgaacagaacgcgctggaaggtatgctggatacgctgaagaaagatatcgccctgggcgaagagttcgttaataagtaa

SEQ ID NO: 32 - protein, 312 aa, Escherichia coli
MKVAVLGAAGGIGQALALLLKTQLPSGSELSLYDIAPVTPGVAVDLSHIPTAVKIKGFSGEDATPALEGADVVLISAGVAAKPGEDRSDLFNVNAGIVKNLVQQVAKTCPKACIGIITNPVNTTVAIAAEVLKKAGVYDKNKLFGVTTLDIIRSNTFVAELKGKQPGEVEVPVIGGHSGVTILPLLSQVPGVSFTEQEVADLTKRIQNAGTEVVEAKAGGGSATLSMGQAAARFGLSLVRALQGEQGVVECAYVEGDGQYARFFSQPLLLGKNGVEERKSIGTLSAFEQNALEGMLDTLKKDIALGEEFVNK

SEQ ID NO: 33 - DNA, 939 bp, Escherichia coli
  source 1..939: mol_type = genomic DNA
atgaaagtcgcagtcctcggcgctgctggcggtgttggccaggcgcttgcactactgttaaaaacccaactgccttcaggttcagaactctctctgtatgatatcgctccagtgactcccggtgtggctgtcgatctgagccatatccctactgctgtgaaaatcaaaggtttttctggtgaagatgcgactccggcgctggaaggcgcagatgtcgttcttatctctgcaggcgtagcggctaaaccgggtcaggatcgttccgacctgtttaacgttaacgccggcatcgtgaaaaacctggtacagcaagttgcgaaaacctgcccgaaagcgtgcattggtattatcactaacccggttaacaccacagttgcaattgctgctgaagtgctgaaaaaagccggtgtttatgacaaaaacaaactgttcggcgttaccacgctggatatcattcgttccaacacctttgttgcggaactgaaaggcaaacagccaggcgaagttgaagtgccggttattggcggtcactctggtgttaccattctgccgctgctgtcacaggttcctggcgttagttttaccgagcaggaagtggctgatctgaccaaacgcatccagaacgcgggtactgaagtggttgaagcgaaggccggtggcgggtctgcaaccctgtctatgggccaggcagctgcacgttttggtctgtctctggttcgtgcactgcagggcgaacaaggcgttgtcgaatgtgcctacgttgaaggcgacggtcagtacgcccgtttcttctctcaaccgctgctgctgggtaaaaacggcgtggaagagcgtaaatctatcggtaccctgagcgcatttgaacagaacgcgctggaaggtatgctggatacgctgaagaaagatatcgccctgggcgaagagttcgttaataagtaa

SEQ ID NO: 34 - protein, 312 aa, Escherichia coli
MKVAVLGAAGGVGQALALLLKTQLPSGSELSLYDIAPVTPGVAVDLSHIPTAVKIKGFSGEDATPALEGADVVLISAGVAAKPGQDRSDLFNVNAGIVKNLVQQVAKTCPKACIGIITNPVNTTVAIAAEVLKKAGVYDKNKLFGVTTLDIIRSNTFVAELKGKQPGEVEVPVIGGHSGVTILPLLSQVPGVSFTEQEVADLTKRIQNAGTEVVEAKAGGGSATLSMGQAAARFGLSLVRALQGEQGVVECAYVEGDGQYARFFSQPLLLGKNGVEERKSIGTLSAFEQNALEGMLDTLKKDIALGEEFVNK

SEQ ID NO: 35 - DNA, 939 bp, Escherichia coli
  source 1..939: mol_type = genomic DNA
atgaaagtcgcagtcctcggcgctgctggcggtgttggccaggcgcttgcactactgttaaaaacccaactgccttcaggttcagaactctctctgtatgatatcgctccagtgactcccggtgtggctgtcgatctgagccatatccctactgctgtgaaaatcaaaggtttttctggtgaagatgcgactccggcgctggaaggcgcagatgtcgttcttatctctgcaggcgtagcggctaaaccgggtgaggatcgttccgacctgtttaacgttaacgccggcatcgtgaaaaacctggtacagcaagttgcgaaaacctgcccgaaagcgtgcattggtattatcactaacccggttaacaccacagttgcaattgctgctgaagtgctgaaaaaagccggtgtttatgacaaaaacaaactgttcggcgttaccacgctggatatcattcgttccaacacctttgttgcggaactgaaaggcaaacagccaggcgaagttgaagtgccggttattggcggtcactctggtgttaccattctgccgctgctgtcacaggttcctggcgttagttttaccgagcaggaagtggctgatctgaccaaacgcatccagaacgcgggtactgaagtggttgaagcgaaggccggtggcgggtctgcaaccctgtctatgggccaggcagctgcacgttttggtctgtctctggttcgtgcactgcagggcgaacaaggcgttgtcgaatgtgcctacgttgaaggcgacggtcagtacgcccgtttcttctctcaaccgctgctgctgggtaaaaacggcgtggaagagcgtaaatctatcggtaccctgagcgcatttgaacagaacgcgctggaaggtatgctggatacgctgaagaaagatatcgccctgggcgaagagttcgttaataagtaa

SEQ ID NO: 36 - protein, 312 aa, Escherichia coli
MKVAVLGAAGGVGQALALLLKTQLPSGSELSLYDIAPVTPGVAVDLSHIPTAVKIKGFSGEDATPALEGADVVLISAGVAAKPGEDRSDLFNVNAGIVKNLVQQVAKTCPKACIGIITNPVNTTVAIAAEVLKKAGVYDKNKLFGVTTLDIIRSNTFVAELKGKQPGEVEVPVIGGHSGVTILPLLSQVPGVSFTEQEVADLTKRIQNAGTEVVEAKAGGGSATLSMGQAAARFGLSLVRALQGEQGVVECAYVEGDGQYARFFSQPLLLGKNGVEERKSIGTLSAFEQNALEGMLDTLKKDIALGEEFVNK

SEQ ID NO: 37 - DNA, 939 bp, Escherichia coli
  source 1..939: mol_type = genomic DNA
atgaaagtcgcagtcctcggcgctgctggcggtattggccaggcgcttgcactactgttaaaaacccaactgccttcaggttcagaactctctctgtatgatatcgctccagtgactcccggtgtggctgtcgatctgagccatatccctactgctgtgaaaatcaaaggtttttctggtgaagatgcgactccggcgctggaaggcgcagatgtcgttcttatctctgcaggcgtagcggctaaaccgggtatggatcgttccgacctgtttaacgttaacgccggcatcgtgaaaaacctggtacagcaagttgcgaaaacctgcccgaaagcgtgcattggtattatcactaacccggttaacaccacagttgcaattgctgctgaagtgctgaaaaaagccggtgtttatgacaaaaacaaactgttcggcgttaccacgctggatatcattcgttccaacacctttgttgcggaactgaaaggcaaacagccaggcgaagttgaagtgccggttattggcggtcactctgatgttaccattctgccgctgctgtcacaggttcctggcgttagttttaccgagcaggaagtggctgatctgaccaaacgcatccagaacgcgggtactgaagtggttgaagcgaaggccggtggcgggtctgcaaccctgtctatgggccaggcagctgcacgttttggtctgtctctggttcgtgcactgcagggcgaacaaggcgttgtcgaatgtgcctacgttgaaggcgacggtcagtacgcccgtttcttctctcaaccgctgctgctgggtaaaaacggcgtggaagagcgtaaatctatcggtaccctgagcgcatttgaacagaacgcgctggaaggtatgctggatacgctgaagaaagatatcgccctgggcgaagagttcgttaataagtaa

SEQ ID NO: 38 - protein, 312 aa, Escherichia coli
MKVAVLGAAGGIGQALALLLKTQLPSGSELSLYDIAPVTPGVAVDLSHIPTAVKIKGFSGEDATPALEGADVVLISAGVAAKPGMDRSDLFNVNAGIVKNLVQQVAKTCPKACIGIITNPVNTTVAIAAEVLKKAGVYDKNKLFGVTTLDIIRSNTFVAELKGKQPGEVEVPVIGGHSDVTILPLLSQVPGVSFTEQEVADLTKRIQNAGTEVVEAKAGGGSATLSMGQAAARFGLSLVRALQGEQGVVECAYVEGDGQYARFFSQPLLLGKNGVEERKSIGTLSAFEQNALEGMLDTLKKDIALGEEFVNK

SEQ ID NO: 39 - DNA, 939 bp, Escherichia coli
  source 1..939: mol_type = genomic DNA
atgaaagtcgcagtcctcggcgctgctggcggtattggccaggcgcttgcactactgttaaaaacccaactgccttcaggttcagaactctctctgtatgatatcgctccagtgactcccggtgtggctgtcgatctgagccatatccctactgctgtgaaaatcaaaggtttttctggtgaagatgcgactccggcgctggaaggcgcagatgtcgttcttatctctgcaggcgtagcggctaaaccgggtatgtctcgttccgacctgtttaacgttaacgccggcatcgtgaaaaacctggtacagcaagttgcgaaaacctgcccgaaagcgtgcattggtattatcactaacccggttaacaccacagttgcaattgctgctgaagtgctgaaaaaagccggtgtttatgacaaaaacaaactgttcggcgttaccacgctggatatcattcgttccaacacctttgttgcggaactgaaaggcaaacagccaggcgaagttgaagtgccggttattggcggtcactctggtgttaccattctgccgctgctgtcacaggttcctggcgttagttttaccgagcaggaagtggctgatctgaccaaacgcatccagaacgcgggtactgaagtggttgaagcgaaggccggtggcgggtctgcaaccctgtctatgggccaggcagctgcacgttttggtctgtctctggttcgtgcactgcagggcgaacaaggcgttgtcgaatgtgcctacgttgaaggcgacggtcagtacgcccgtttcttctctcaaccgctgctgctgggtaaaaacggcgtggaagagcgtaaatctatcggtaccctgagcgcatttgaacagaacgcgctggaaggtatgctggatacgctgaagaaagatatcgccctgggcgaagagttcgttaataagtaa

SEQ ID NO: 40 - protein, 312 aa, Escherichia coli
MKVAVLGAAGGIGQALALLLKTQLPSGSELSLYDIAPVTPGVAVDLSHIPTAVKIKGFSGEDATPALEGADVVLISAGVAAKPGMSRSDLFNVNAGIVKNLVQQVAKTCPKACIGIITNPVNTTVAIAAEVLKKAGVYDKNKLFGVTTLDIIRSNTFVAELKGKQPGEVEVPVIGGHSGVTILPLLSQVPGVSFTEQEVADLTKRIQNAGTEVVEAKAGGGSATLSMGQAAARFGLSLVRALQGEQGVVECAYVEGDGQYARFFSQPLLLGKNGVEERKSIGTLSAFEQNALEGMLDTLKKDIALGEEFVNK

SEQ ID NO: 41 - DNA, 939 bp, Escherichia coli
  source 1..939: mol_type = genomic DNA
atgaaagtcgcagtcctcggcgctgctggcggtgttggccaggcgcttgcactactgttaaaaacccaactgccttcaggttcagaactctctctgtatgatatcgctccagtgactcccggtgtggctgtcgatctgagccatatccctactgctgtgaaaatcaaaggtttttctggtgaagatgcgactccggcgctggaaggcgcagatgtcgttcttatctctgcaggcgtagcggctaaaccgggtatggatcgttccgacctgtttaacgttaacgccggcatcgtgaaaaacctggtacagcaagttgcgaaaacctgcccgaaagcgtgcattggtattatcactaacccggttaacaccacagttgcaattgctgctgaagtgctgaaaaaagccggtgtttatgacaaaaacaaactgttcggcgttaccacgctggatatcattcgttccaacacctttgttgcggaactgaaaggcaaacagccaggcgaagttgaagtgccggttattggcggtcactctggtgttaccattctgccgctgctgtcacaggttcctggcgttagttttaccgagcaggaagtggctgatctgaccaaacgcatccagaacgcgggtactgaagtggttgaagcgaaggccggtggcgggtctgcaaccctgtctatgggccaggcagctgcacgttttggtctgtctctggttcgtgcactgcagggcgaacaaggcgttgtcgaatgtgcctacgttgaaggcgacggtcagtacgcccgtttcttctctcaaccgctgctgctgggtaaaaacggcgtggaagagcgtaaatctatcggtaccctgagcgcatttgaacagaacgcgctggaaggtatgctggatacgctgaagaaagatatcgccctgggcgaagagttcgttaataagtaa

SEQ ID NO: 42 - protein, 312 aa, Escherichia coli
MKVAVLGAAGGVGQALALLLKTQLPSGSELSLYDIAPVTPGVAVDLSHIPTAVKIKGFSGEDATPALEGADVVLISAGVAAKPGMDRSDLFNVNAGIVKNLVQQVAKTCPKACIGIITNPVNTTVAIAAEVLKKAGVYDKNKLFGVTTLDIIRSNTFVAELKGKQPGEVEVPVIGGHSGVTILPLLSQVPGVSFTEQEVADLTKRIQNAGTEVVEAKAGGGSATLSMGQAAARFGLSLVRALQGEQGVVECAYVEGDGQYARFFSQPLLLGKNGVEERKSIGTLSAFEQNALEGMLDTLKKDIALGEEFVNK

SEQ ID NO: 43 - DNA, 939 bp, Escherichia coli
  source 1..939: mol_type = genomic DNA
atgaaagtcgcagtcctcggcgctgctggcggtattggccaggcgcttgcactactgttaaaaacccaactgccttcaggttcagaactctctctgtatgatatcgctccagtgactcccggtgtggctgtcgatctgagccatatccctactgctgtgaaaatcaaaggtttttctggtgaagatgcgactccggcgctggaaggcgcagatgtcgttcttatctctgcaggcgtagcggctaaaccgggtatgtctcgttccgacctgtttaacgttaacgccggcatcgtgaaaaacctggtacagcaagttgcgaaaacctgcccgaaagcgtgcattggtattatcactaacccggttaacaccacagttgcaattgctgctgaagtgctgaaaaaagccggtgtttatgacaaaaacaaactgttcggcgttaccacgctggatatcattcgttccaacacctttgttgcggaactgaaaggcaaacagccaggcgaagttgaagtgccggttattggcggtcactctgatgttaccattctgccgctgctgtcacaggttcctggcgttagttttaccgagcaggaagtggctgatctgaccaaacgcatccagaacgcgggtactgaagtggttgaagcgaaggccggtggcgggtctgcaaccctgtctatgggccaggcagctgcacgttttggtctgtctctggttcgtgcactgcagggcgaacaaggcgttgtcgaatgtgcctacgttgaaggcgacggtcagtacgcccgtttcttctctcaaccgctgctgctgggtaaaaacggcgtggaagagcgtaaatctatcggtaccctgagcgcatttgaacagaacgcgctggaaggtatgctggatacgctgaagaaagatatcgccctgggcgaagagttcgttaataagtaa

SEQ ID NO: 44 - protein, 312 aa, Escherichia coli
MKVAVLGAAGGIGQALALLLKTQLPSGSELSLYDIAPVTPGVAVDLSHIPTAVKIKGFSGEDATPALEGADVVLISAGVAAKPGMSRSDLFNVNAGIVKNLVQQVAKTCPKACIGIITNPVNTTVAIAAEVLKKAGVYDKNKLFGVTTLDIIRSNTFVAELKGKQPGEVEVPVIGGHSDVTILPLLSQVPGVSFTEQEVADLTKRIQNAGTEVVEAKAGGGSATLSMGQAAARFGLSLVRALQGEQGVVECAYVEGDGQYARFFSQPLLLGKNGVEERKSIGTLSAFEQNALEGMLDTLKKDIALGEEFVNK

SEQ ID NO: 45 - DNA, 939 bp, Escherichia coli; identical to SEQ ID NO: 19
  source 1..939: mol_type = genomic DNA

SEQ ID NO: 46 - protein, 312 aa, Escherichia coli; identical to SEQ ID NO: 20

SEQ ID NO: 47 - DNA, 990 bp, Escherichia coli
  source 1..990: mol_type = genomic DNA
atgaaactcgccgtttatagcacaaaacagtacgacaagaagtacctgcaacaggtgaacgagtcctttggctttgagctggaattttttgactttctgctgacggaaaaaaccgctaaaactgccaatggctgcgaagcggtatgtattttcgtaaacgatgacggcagccgcccggtgctggaagagctgaaaaagcacggcgttaaatatatcgccctgcgctgtgccggtttcaataacgtcgaccttgacgcggcaaaagaactggggctgaaagtagtccgtgttccagcctatgatccagaggccgttgctgaacacgccatcggtatgatgatgacgctgaaccgccgtattcaccgcgcgtatcagcgtacccgtgatgctaacttctctctggaaggtctgaccggctttactatgtatggcaaaacggcaggcgttatcggtaccggtaaaatcggtgtggcgatgctgcgcattctgaaaggttttggtatgcgtctgctggcgttcgatccgtatccaagtgcagcggcgctggaactcggtgtggagtatgtcgatctgccaaccctgttctctgaatcagacgttatctctctgcactgcccgctgacaccggaaaactatcatctgttgaacgaagccgccttcgaacagatgaaaaatggcgtgatgatcgtcaataccagtcgcggtgcattgattgattctcaggcagcaattgaagcgctgaaaaatcagaaaattggttcgttgggtatggacgtgtatgagaacgaacgcgatctattctttgaagataaatccaacgacgtgatccaggatgacgtattccgtcgcctgtctgcctgccacaacgtgctgtttaccgggcaccaggcattcctgacagcagaagctctgaccagtatttctcagactacgctgcaaaacttaagcaatctggaaaaaggcgaaacctgcccgaacgaactggtttaa

SEQ ID NO: 48 - protein, 329 aa, Escherichia coli
MKLAVYSTKQYDKKYLQQVNESFGFELEFFDFLLTEKTAKTANGCEAVCIFVNDDGSRPVLEELKKHGVKYIALRCAGFNNVDLDAAKELGLKVVRVPAYDPEAVAEHAIGMMMTLNRRIHRAYQRTRDANFSLEGLTGFTMYGKTAGVIGTGKIGVAMLRILKGFGMRLLAFDPYPSAAALELGVEYVDLPTLFSESDVISLHCPLTPENYHLLNEAAFEQMKNGVMIVNTSRGALIDSQAAIEALKNQKIGSLGMDVYENERDLFFEDKSNDVIQDDVFRRLSACHNVLFTGHQAFLTAEALTSISQTTLQNLSNLEKGETCPNELV

SEQ ID NO: 49 - DNA, 978 bp, Lactococcus lactis
  source 1..978: mol_type = genomic DNA
atggctgataaacaacgtaaaaaagttatccttgtaggtgacggtgctgtaggttcatcatacgcttttgctcttgtaaaccaagggattgcacaagaattaggaattgttgacctttttaaagaaaaaactcaaggagatgcagaagacctttctcatgccttggcatttacttcacctaaaaagatttactctgcagactactctgatgcaagcgacgctgacctcgtagtcttgacttctggtgctccacaaaaaccaggtgaaactcgtcttgaccttgttgaaaaaaatcttcgtatcactaaagatgttgtcactaaaattgttgcttcaggtttcaaaggaatcttccttgttgctgctaacccagttgatatcttgacatacgctacttggaaattctcaggtttccctaaaaaccgcgttgtaggttcaggtacttcacttgatactgcacgtttccgtcaagcattggcagaaaaagttgatgttgacgctcgttcaatccacgcatacatcatgggtgaacacggtgactcagaatttgccgtttggtcacacgctaacgttgctggtgttaaattggaacaatggttccaagaaaatgactaccttaacgaagctgaaatcgttgaattgtttgaatctgtacgtgatgctgcttactcaatcatcgctaaaaaaggtgcaacattctatggtgtcgctgtagctcttgctcgtattactaaagcaattcttgatgatgaacatgcagtacttccagtatcagtattccaagatggacaatatggcgtaagcgactgctaccttggtcaaccagctgtagttggtgctgaaggtgttgttaacccaatccacattccattgaatgatgctgaaatgcaaaaaatggaagcttctggtgctcaattgaaagcaatcattgacgaagcttttgctaaagaagaatttgcttctgcagttaaaaactaa

SEQ ID NO: 50 - protein, 325 aa, Lactococcus lactis
MADKQRKKVILVGDGAVGSSYAFALVNQGIAQELGIVDLFKEKTQGDAEDLSHALAFTSPKKIYSADYSDASDADLVVLTSGAPQKPGETRLDLVEKNLRITKDVVTKIVASGFKGIFLVAANPVDILTYATWKFSGFPKNRVVGSGTSLDTARFRQALAEKVDVDARSIHAYIMGEHGDSEFAVWSHANVAGVKLEQWFQENDYLNEAEIVELFESVRDAAYSIIAKKGATFYGVAVALARITKAILDDEHAVLPVSVFQDGQYGVSDCYLGQPAVVGAEGVVNPIHIPLNDAEMQKMEASGAQLKAIIDEAFAKEEFASAVKN

SEQ ID NO: 51 - DNA, 966 bp, Bacillus subtilis
  source 1..966: mol_type = genomic DNA
atgatgaacaaacatgtaaataaagtagctttaatcggagcgggttttgttggaagcagttatgcatttgcgttaattaaccaaggaatcacagatgagcttgtggtcattgatgtaaataaagaaaaagcaatgggcgatgtgatggatttaaaccacggaaaggcgtttgcgccacaaccggtcaaaacatcttacggaacatatgaagactgcaaggatgctgatattgtctgcatttgcgccggagcaaaccaaaaacctggtgagacacgccttgaattagtagaaaagaacttgaagattttcaaaggcatcgttagtgaagtcatggcgagcggatttgacggcattttcttagtcgcgacaaatccggttgatatcctgacttacgcaacatggaaattcagcggcctgccaaaagagcgggtgattggaagcggcacaacacttgattctgcgagattccgtttcatgctgagcgaatactttggcgcagcgcctcaaaacgtacacgcgcatattatcggagagcacggcgacacagagcttcctgtttggagccacgcgaatgtcggcggtgtgccggtcagtgaactcgttgagaaaaacgatgcgtacaaacaagaggagctggaccaaattgtagatgatgtgaaaaacgcagcttaccatatcattgagaaaaaaggcgcgacttattatggggttgcgatgagtcttgctcgcattacaaaagccattcttcataatgaaaacagcatattaactgtcagcacatatttggacgggcaatacggtgcagatgacgtgtacatcggtgtgccggctgtcgtgaatcgcggagggatcgcaggtatcactgagctgaacttaaatgagaaagaaaaagaacagttccttcacagcgccggcgtccttaaaaacattttaaaacctcattttgcagaacaaaaagtcaactaa

SEQ ID NO: 52 - protein, 321 aa, Bacillus subtilis
MMNKHVNKVALIGAGFVGSSYAFALINQGITDELVVIDVNKEKAMGDVMDLNHGKAFAPQPVKTSYGTYEDCKDADIVCICAGANQKPGETRLELVEKNLKIFKGIVSEVMASGFDGIFLVATNPVDILTYATWKFSGLPKERVIGSGTTLDSARFRFMLSEYFGAAPQNVHAHIIGEHGDTELPVWSHANVGGVPVSELVEKNDAYKQEELDQIVDDVKNAAYHIIEKKGATYYGVAMSLARITKAILHNENSILTVSTYLDGQYGADDVYIGVPAVVNRGGIAGITELNLNEKEKEQFLHSAGVLKNILKPHFAEQKVN

SEQ ID NO: 53 - DNA, 954 bp, Geobacillus stearothermophilus
  source 1..954: mol_type = genomic DNA
atgaagaacaatggtggagcgcgtgttgtggtaattggcgcgggttttgtgggtgccagctatgttttcgcgttaatgaaccaaggtattgcagacgagattgtcctgattgacgcgaatgaatccaaagcgattggggacgccatggatttcaaccacggtaaagtgtttgctccgaaaccggtcgatatctggcatggcgattacgacgattgtcgcgatgccgatctggtggtcatctgcgctggtgcaaaccagaaacccggtgaaactcgtctggatcttgttgacaagaacattgccatctttcggtctattgtcgaaagcgtgatggcaagtgggtttcagggactgtttctggttgccaccaatccggtagacatcctgacgtatgctacctggaaattcagcggcttaccgcatgaacgtgttatcggcagtggtaccattcttgatacggcacgttttcgcttcctgttgggagagtacttctccgttgcccctcagaatgtgcatgcctacatcattggggaacatggcgataccgaattgccagtgtggtcgcaagcgtatattggtgtaatgccgattcgcaaactggtggaatcgaaaggcgaagaagcccagaaagacttggaacgcatctttgtcaacgtacgcgatgcagcgtatcagatcatcgagaaaaaaggtgcgacctattacggcatcgcaatgggcttagctcgtgtaactcgggctattctgcacaacgagaacgcgattctcacagtgtcagcgtatctcgatgggctgtatggcgaacgcgatgtgtacattggcgttccagccgtcatcaatcgcaatggcattcgtgaggtgattgaaatcgaactgaacgatgacgagaagaatcgcttccatcactctgcggctacactgaaaagcgttctcgcacgtgcgtttacgcgctaa

SEQ ID NO: 54 - protein, 317 aa, Geobacillus stearothermophilus
MKNNGGARVVVIGAGFVGASYVFALMNQGIADEIVLIDANESKAIGDAMDFNHGKVFAPKPVDIWHGDYDDCRDADLVVICAGANQKPGETRLDLVDKNIAIFRSIVESVMASGFQGLFLVATNPVDILTYATWKFSGLPHERVIGSGTILDTARFRFLLGEYFSVAPQNVHAYIIGEHGDTELPVWSQAYIGVMPIRKLVESKGEEAQKDLERIFVNVRDAAYQIIEKKGATYYGIAMGLARVTRAILHNENAILTVSAYLDGLYGERDVYIGVPAVINRNGIREVIEIELNDDEKNRFHHSAATLKSVLARAFTR

SEQ ID NO: 55 - DNA, 999 bp, Oryctolagus cuniculus
  source 1..999: mol_type = genomic DNA
atggcggcgttgaaagaccaactgattcataaccttttaaaagaggaacatgtgccgcagaacaaaattaccgttgtaggcgtaggtgcagttggtatggcctgtgccattagcatcctgatgaaagacttggcggatgaacttgctctggtcgatgtaatggaggataaactgaaaggcgaaatgatggacttgcagcatgggtcgctgtttcttcgcacacccaagatcgtaagcggcaaagattactccgtgactgcaaattccaaattggtcatcattaccgccggagcacgccagcaagaaggtgaaagccgcctgaacctggtgcaacggaacgtcaacattttcaaatttatcattccgaacgtggtgaaatactctccacactgcaaactcctcgttgttagtaaccctgttgacatcctgacgtatgttgcctggaaaattagcggcttcccgaagaatcgcgtaattggctcaggatgcaatctggattcggcgcgttttcgctatctgatgggcgaacgtttaggtgttcatgcactgtcatgccacgggtggattctgggtgaacatggcgatagttctgtgcctgtgtggtctggcatgaatgtggctggtgtgtcactgaaaacgttacacccagaacttggcactgacgcggataaagagcagtggaaacaggtacacaaacaggtggtcgatagcgcgtatgaggtcatcaaactgaaaggttacaccacatgggccattgggctgagtgtcgccgatctggctgagagcattatgaagaatctccgtcgtgttcatccgatctccacgatgctcaaaggtctgtatgggatcaaagaggacgttttcttaagtgtgccgtgtgtcctgggtcagaatggcatttcggatgtggtcaaggtgaccttaacctcggaagaagaagcgcacctgaagaagagcgcggataccttgtggggaatccagaaagaactgcaattttaa

SEQ ID NO: 56 - protein, 332 aa, Oryctolagus cuniculus
MAALKDQLIHNLLKEEHVPQNKITVVGVGAVGMACAISILMKDLADELALVDVMEDKLKGEMMDLQHGSLFLRTPKIVSGKDYSVTANSKLVIITAGARQQEGESRLNLVQRNVNIFKFIIPNVVKYSPHCKLLVVSNPVDILTYVAWKISGFPKNRVIGSGCNLDSARFRYLMGERLGVHALSCHGWILGEHGDSSVPVWSGMNVAGVSLKTLHPELGTDADKEQWKQVHKQVVDSAYEVIKLKGYTTWAIGLSVADLAESIMKNLRRVHPISTMLKGLYGIKEDVFLSVPCVLGQNGISDVVKVTLTSEEEAHLKKSADTLWGIQKELQF

SEQ ID NO: 57 - DNA, 1014 bp, Oryctolagus cuniculus
  source 1..1014: mol_type = genomic DNA
atggcaacgctgaaagagaaattgatcgcacctgtcgccgataacgaagcggctgttccgaacaacaaaattaccgtagtaggcgtcggtcaagtaggcatggcgtgtgcgatttccattctcggcaaaagtttagcggacgaactggcacttgtcgatgtcttggaagataaactgaaaggtgaaatgatggatttacagcatggttcgctgtttctccagacacccaaaattgtggcggataaagattacagtgtgactgcgaacagcaagatcgtagttgtcaccgccggagtccgtcaacaggaaggtgaatcacgcctgaacttggtgcaacgcaatgtgaatgtgttcaaattcatcatcccgcagattgttaagtatagcccgaactgcatcatcattgtcgtcagcaaccctgagtgtctggttgacatcctgacgtacgttacctggaaactctccggactgccgaaacaccgcgtaattggctcgggttgcaatctggacagcgctcgttttcggtatcttatggccgagaaattaggtattcacccatctagttgtcatggatggattctgggtgaacatggcgatagctctgtggcagtatggtctggcgttaacgttgcgggtgtgtcgttgcaagaactgaatccggagatggggaccgataatgatagcgaaaattggaaagaggtgcacaaaatggtggtggaaagcgcctatgaagtgattaagctgaaagggtacaccaactgggcaattggcttatcagttgcggatcttatcgagtccatgctgaagaatctgtcacgcattcatccggtttccacaatggtgaaaggcatgtatgggatcgaaaacgaagtgtttctgtctttaccatgcatcctgaatgctcgtggcctcacttcggtgattaatcagaagctgaaagatgacgaagttgcccagctgaagaaaagtgccgatacgctgtgggacattcagaaagacctgaaagacctttaa

SEQ ID NO: 58 - protein, 337 aa, Oryctolagus cuniculus
MATLKEKLIAPVADNEAAVPNNKITVVGVGQVGMACAISILGKSLADELALVDVLEDKLKGEMMDLQHGSLFLQTPKIVADKDYSVTANSKIVVVTAGVRQQEGESRLNLVQRNVNVFKFIIPQIVKYSPNCIIIVVSNPECLVDILTYVTWKLSGLPKHRVIGSGCNLDSARFRYLMAEKLGIHPSSCHGWILGEHGDSSVAVWSGVNVAGVSLQELNPEMGTDNDSENWKEVHKMVVESAYEVIKLKGYTNWAIGLSVADLIESMLKNLSRIHPVSTMVKGMYGIENEVFLSLPCILNARGLTSVINQKLKDDEVAQLKKSADTLWDIQKDLKDL

SEQ ID NO: 59 - DNA, 939 bp, Lactococcus lactis
  source 1..939: mol_type = genomic DNA
atgagaattacaattgccggtgcaggagcgatggggagtcgttttggtttaatgcttcataaaggtggcaatgaagtaacccttatagatggatggcctgaacacgttaaagcgattaaagagcatggtttgcgagctaattacaatggagaagaactcaccgctcatctatcggttgagttacaatctgagatttcttctaaagaaaaaacagatttaattattttgtttacaaaagccatgcaattagataagatgctacaagatattaaaccattaattgacgagcataccaaggtactttgcttactaaatggaattggtcacgaagatactatagaaaaatatgtttcgaaaaataatatctttattggtaatactatgtggactgctggattagaaggtccaggtaaagctaaattatttggtgatggttcggttgagctacaaaatcttatttcaggtgaggaagaaacagctaaaaagttagcagaaatattatcagaatcgggactgaatgctaaatattctaacaatattcattattctatttatagaaaagcttgtgttaatggaacaatgaatgggctttgtactattttagacactaatatggccggattaggtgaaacaaaaccagcacatgatatggttgttactattgttaatgaatttgcagcagtagcaaaatttgagaatgtaaaccttgatattgctgaagtagttcagcacgttgaaacatgttttgatccatctacaattggattacattacccttctatgtatcaggatttgattaaaaataatcgattgacagagattgactatattaatggggctgtttcacgtaaaggtaaaaaatataatgtagccacaccttattgtgatttcttaacacaattagttcacagcaaagaagagttattaaaagcaaaataa

SEQ ID NO: 60 - protein, 312 aa, Lactococcus lactis
MRITIAGAGAMGSRFGLMLHKGGNEVTLIDGWPEHVKAIKEHGLRANYNGEELTAHLSVELQSEISSKEKTDLIILFTKAMQLDKMLQDIKPLIDEHTKVLCLLNGIGHEDTIEKYVSKNNIFIGNTMWTAGLEGPGKAKLFGDGSVELQNLISGEEETAKKLAEILSESGLNAKYSNNIHYSIYRKACVNGTMNGLCTILDTNMAGLGETKPAHDMVVTIVNEFAAVAKFENVNLDIAEVVQHVETCFDPSTIGLHYPSMYQDLIKNNRLTEIDYINGAVSRKGKKYNVATPYCDFLTQLVHSKEELLKAK

SEQ ID NO: 61 - DNA, 978 bp, Lactococcus lactis
  source 1..978: mol_type = genomic DNA
atggctgataaacaacgtaaaaaagttatccttgtaggtgacggtgctgtaggttcatcatacgcttttgctcttgtaaaccaagggattgcacaagaattaggaattgttgacctttttaaagaaaaaactcaaggagatgcagaagacctttctcatgccttggcatttacttcacctaaaaagatttactctgcagactactctgatgcaagcgacgctgacctcgtagtcttgacgtctggtgctccaaataaaccaggtgaaactcgtcttgaccttgttgaaaaaaatcttcgtatcactaaagatgttgtcactaaaattgttgcttcaggtttcaaaggaatcttccttgttgctgctaacccagttgatatcttgacatacgctacttggaaattctcaggtttccctaaaaaccgcgttgtaggttcaggtacttcacttgatactgcacgtttccgtcaagcattggcagaaaaagttgatgttgacgctcgttcaatccacgcatacatcatgggtgaacacggtgactcagaatttgccgtttggtcacacgctaacgttgctggtgttaaattggaacaatggttccaagaaaatgactaccttaacgaagctgaaatcgttgaattgtttgaatctgtacgtgatgctgcttactcaatcatcgctaaaaaaggtgcaacattctatggtgtcgctgtagctcttgctcgtattactaaagcaattcttgatgatgaacatgcagtacttccagtatcagtattccaagatggacaatatggcgtaagcgactgctaccttggtcaaccagctgtagttggtgctgaaggtgttgttaacccaatccacattccattgaatgatgctgaaatgcaaaaaatggaagcttctggtgctcaattgaaagcaatcattgacgaagcttttgctaaagaagaatttgcttctgcagttaaaaactaa

SEQ ID NO: 62 - protein, 325 aa, Lactococcus lactis
MADKQRKKVILVGDGAVGSSYAFALVNQGIAQELGIVDLFKEKTQGDAEDLSHALAFTSPKKIYSADYSDASDADLVVLTSGAPNKPGETRLDLVEKNLRITKDVVTKIVASGFKGIFLVAANPVDILTYATWKFSGFPKNRVVGSGTSLDTARFRQALAEKVDVDARSIHAYIMGEHGDSEFAVWSHANVAGVKLEQWFQENDYLNEAEIVELFESVRDAAYSIIAKKGATFYGVAVALARITKAILDDEHAVLPVSVFQDGQYGVSDCYLGQPAVVGAEGVVNPIHIPLNDAEMQKMEASGAQLKAIIDEAFAKEEFASAVKN

SEQ ID NO: 63 - DNA, 978 bp, Lactococcus lactis
  source 1..978: mol_type = genomic DNA
atggctgataaacaacgtaaaaaagttatccttgtaggtgacggtgctgtaggttcatcatacgcttttgctcttgtaaaccaagggattgcacaagaattaggaattgttgacctttttaaagaaaaaactcaaggagatgcagaagacctttctcatgccttggcatttacttcacctaaaaagatttactctgcagactactctgatgcaagcgacgctgacctcgtagtcttgacgtctggtgctccaaataaaccaggtgaaactcgtcttgaccttgttgaaaaaaatcttcgtatcactaaagatgttgtcactaaaattgttgcttcaggtttcaaaggaatcttccttgttgctgctaacccagttgatatcttgacatacgctacttggaaattctcaggtttccctaaaaaccgcgttgtaggttcaggtacttcacttgatactgcacgtttccgtcaagcattggcagaaaaagttgatgttgacgctcgttcaatccacgcatacatcatgggtgaacacggtgactcagaatttgccgtttggtcacacgctaacgttgctggtgttaaattggaacaatggttccaagaaaatgactaccttaacgaagctgaaatcgttgaattgtttgaatctgtacgtgatgctgcttactcgatcgtcgctaaaaaaggtgcaacattctatggtgtcgctgtagctcttgctcgtattactaaagcaattcttgatgatgaacatgcagtacttccagtatcagtattccaagatggacaatatggcgtaagcgactgctaccttggtcaaccagctgtagttggtgctgaaggtgttgttaacccaatccacattccattgaatgatgctgaaatgcaaaaaatggaagcttctggtgctcaattgaaagcaatcattgacgaagcttttgctaaagaagaatttgcttctgcagttaaaaactaa

SEQ ID NO: 64 - protein, 325 aa, Lactococcus lactis
MADKQRKKVILVGDGAVGSSYAFALVNQGIAQELGIVDLFKEKTQGDAEDLSHALAFTSPKKIYSADYSDASDADLVVLTSGAPNKPGETRLDLVEKNLRITKDVVTKIVASGFKGIFLVAANPVDILTYATWKFSGFPKNRVVGSGTSLDTARFRQALAEKVDVDARSIHAYIMGEHGDSEFAVWSHANVAGVKLEQWFQENDYLNEAEIVELFESVRDAAYSIVAKKGATFYGVAVALARITKAILDDEHAVLPVSVFQDGQYGVSDCYLGQPAVVGAEGVVNPIHIPLNDAEMQKMEASGAQLKAIIDEAFAKEEFASAVKN

SEQ ID NO: 65 - DNA, 939 bp, Escherichia coli
  source 1..939: mol_type = genomic DNA
atgaaagtcgcagtcctcggcgctgctggcggtattggccaggcgcttgcactactgttaaaaacccaactgccttcaggttcagaactctctctgtatgatatcgctccagtgactcccggtgtggctgtcgatctgagccatatccctactgctgtgaaaatcaaaggtttttctggtgaagatgcgactccggcgctggaaggcgcagatgtcgttcttatctctgcaggcgtagcggctaaacccgggatggatcgttccgacctgtttaacgttaacgccggcatcgtgaaaaacctggtacagcaagttgcgaaaacctgcccgaaagcgtgcattggtattatcactaacccggttaacaccacagttgcaattgctgctgaagtgctgaaaaaagccggtgtttatgacaaaaacaaactgttcggcgttaccacgctggatatcattcgttccaacacctttgttgcggaactgaaaggcaaacagccaggcgaagttgaagtgccggttattggcggtcactctggtgttaccattctgccgctgctgtcacaggttcctggcgttagttttaccgagcaggaagtggctgatctgaccaaacgcatccagaacgcgggtactgaagtggttgaagcgaaggccggtggcgggtctgcaaccctgtctatgggccaggcagctgcacgttttggtctgtctctggttcgtgcactgcagggcgaacaaggcgttgtcgaatgtgcctacgttgaaggcgacggtcagtacgcccgtttcttctctcaaccgctgctgctgggtaaaaacggcgtggaagagcgtaaatctatcggtaccctgagcgcatttgaacagaacgcgctggaaggtatgctggatacgctgaagaaagatatcgccctgggcgaagagttcgttaataagtaa

SEQ ID NO: 66 - protein, 312 aa, Escherichia coli; identical to SEQ ID NO: 28

SEQ ID NO: 67 - DNA, 939 bp, Escherichia coli; identical to SEQ ID NO: 29
  source 1..939: mol_type = genomic DNA

SEQ ID NO: 68 - protein, 312 aa, Escherichia coli; identical to SEQ ID NO: 30

SEQ ID NO: 69 - DNA, 939 bp, Escherichia coli; identical to SEQ ID NO: 31
  source 1..939: mol_type = genomic DNA

SEQ ID NO: 70 - protein, 312 aa, Escherichia coli; identical to SEQ ID NO: 32

SEQ ID NO: 71 - DNA, 939 bp, Escherichia coli
  source 1..939: mol_type = genomic DNA
atgaaagtcgcagtcctcggcgccgctggcggtgtcggccaggcgcttgcactactgttaaaaacccaactgccttcaggttcagaactctctctgtatgatatcgctccagtgactcccggtgtggctgtcgatctgagccatatccctactgctgtgaaaatcaaaggtttttctggtgaagatgcgactccggcgctggaaggcgcagatgtcgttcttatctctgcaggcgtagcggctaaaccgggtcaggatcgttccgacctgtttaacgttaacgccggcatcgtgaaaaacctggtacagcaagttgcgaaaacctgcccgaaagcgtgcattggtattatcactaacccggttaacaccacagttgcaattgctgctgaagtgctgaaaaaagccggtgtttatgacaaaaacaaactgttcggcgttaccacgctggatatcattcgttccaacacctttgttgcggaactgaaaggcaaacagccaggcgaagttgaagtgccggttattggcggtcactctggtgttaccattctgccgctgctgtcacaggttcctggcgttagttttaccgagcaggaagtggctgatctgaccaaacgcatccagaacgcgggtactgaagtggttgaagcgaaggccggtggcgggtctgcaaccctgtctatgggccaggcagctgcacgttttggtctgtctctggttcgtgcactgcagggcgaacaaggcgttgtcgaatgtgcctacgttgaaggcgacggtcagtacgcccgtttcttctctcaaccgctgctgctgggtaaaaacggcgtggaagagcgtaaatctatcggtaccctgagcgcatttgaacagaacgcgctggaaggtatgctggatacgctgaagaaagatatcgccctgggcgaagagttcgttaataagtaa

SEQ ID NO: 72 - protein, 312 aa, Escherichia coli; identical to SEQ ID NO: 34

SEQ ID NO: 73 - DNA, 939 bp, Escherichia coli
  source 1..939: mol_type = genomic DNA
atgaaagtcgcagtcctcggcgccgctggcggtgtcggccaggcgcttgcactactgttaaaaacccaactgccttcaggttcagaactctctctgtatgatatcgctccagtgactcccggtgtggctgtcgatctgagccatatccctactgctgtgaaaatcaaaggtttttctggtgaagatgcgactccggcgctggaaggcgcagatgtcgttcttatctctgcaggcgtagcggctaaaccgggtgaggatcgttccgacctgtttaacgttaacgccggcatcgtgaaaaacctggtacagcaagttgcgaaaacctgcccgaaagcgtgcattggtattatcactaacccggttaacaccacagttgcaattgctgctgaagtgctgaaaaaagccggtgtttatgacaaaaacaaactgttcggcgttaccacgctggatatcattcgttccaacacctttgttgcggaactgaaaggcaaacagccaggcgaagttgaagtgccggttattggcggtcactctggtgttaccattctgccgctgctgtcacaggttcctggcgttagttttaccgagcaggaagtggctgatctgaccaaacgcatccagaacgcgggtactgaagtggttgaagcgaaggccggtggcgggtctgcaaccctgtctatgggccaggcagctgcacgttttggtctgtctctggttcgtgcactgcagggcgaacaaggcgttgtcgaatgtgcctacgttgaaggcgacggtcagtacgcccgtttcttctctcaaccgctgctgctgggtaaaaacggcgtggaagagcgtaaatctatcggtaccctgagcgcatttgaacagaacgcgctggaaggtatgctggatacgctgaagaaagatatcgccctgggcgaagagttcgttaataagtaa

SEQ ID NO: 74 - protein, 312 aa, Escherichia coli; identical to SEQ ID NO: 36

SEQ ID NO: 75 - DNA, 939 bp, Escherichia coli
  source 1..939: mol_type = genomic DNA
atgaaagtcgcagtcctcggcgctgctggcggtattggccaggcgcttgcactactgttaaaaacccaactgccttcaggttcagaactctctctgtatgatatcgctccagtgactcccggtgtggctgtcgatctgagccatatccctactgctgtgaaaatcaaaggtttttctggtgaagatgcgactccggcgctggaaggcgcagatgtcgttcttatctctgcaggcgtagcggctaaacccgggatggatcgttccgacctgtttaacgttaacgccggcatcgtgaaaaacctggtacagcaagttgcgaaaacctgcccgaaagcgtgcattggtattatcactaacccggttaacaccacagttgcaattgctgctgaagtgctgaaaaaagccggtgtttatgacaaaaacaaactgttcggcgttaccacgctggatatcattcgttccaacacctttgttgcggaactgaaaggcaaacagccaggcgaagttgaagtgccggttattggcggccactctgatgttaccattctgccgctgctgtcacaggttcctggcgttagttttaccgagcaggaagtggctgatctgaccaaacgcatccagaacgcgggtactgaagtggttgaagcgaaggccggtggcgggtctgcaaccctgtctatgggccaggcagctgcacgttttggtctgtctctggttcgtgcactgcagggcgaacaaggcgttgtcgaatgtgcctacgttgaaggcgacggtcagtacgcccgtttcttctctcaaccgctgctgctgggtaaaaacggcgtggaagagcgtaaatctatcggtaccctgagcgcatttgaacagaacgcgctggaaggtatgctggatacgctgaagaaagatatcgccctgggcgaagagttcgttaataagtaa

SEQ ID NO: 76 - protein, 312 aa, Escherichia coli; identical to SEQ ID NO: 38

SEQ ID NO: 77 - DNA, 939 bp, Escherichia coli
  source 1..939: mol_type = genomic DNA
atgaaagtcgcagtcctcggcgctgctggcggtattggccaggcgcttgcactactgttaaaaacccaactgccttcaggttcagaactctctctgtatgatatcgctccagtgactcccggtgtggctgtcgatctgagccatatccctactgctgtgaaaatcaaaggtttttctggtgaagatgcgactccggcgctggaaggcgcagatgtcgttcttatctctgcaggcgtagcggctaaacccgggatgtctcgttccgacctgtttaacgttaacgccggcatcgtgaaaaacctggtacagcaagttgcgaaaacctgcccgaaagcgtgcattggtattatcactaacccggttaacaccacagttgcaattgctgctgaagtgctgaaaaaagccggtgtttatgacaaaaacaaactgttcggcgttaccacgctggatatcattcgttccaacacctttgttgcggaactgaaaggcaaacagccaggcgaagttgaagtgccggttattggcggtcactctggtgttaccattctgccgctgctgtcacaggttcctggcgttagttttaccgagcaggaagtggctgatctgaccaaacgcatccagaacgcgggtactgaagtggttgaagcgaaggccggtggcgggtctgcaaccctgtctatgggccaggcagctgcacgttttggtctgtctctggttcgtgcactgcagggcgaacaaggcgttgtcgaatgtgcctacgttgaaggcgacggtcagtacgcccgtttcttctctcaaccgctgctgctgggtaaaaacggcgtggaagagcgtaaatctatcggtaccctgagcgcatttgaacagaacgcgctggaaggtatgctggatacgctgaagaaagatatcgccctgggcgaagagttcgttaataagtaa

SEQ ID NO: 78 - protein, 312 aa, Escherichia coli; identical to SEQ ID NO: 40

SEQ ID NO: 79 - DNA, 939 bp, Escherichia coli
  source 1..939: mol_type = genomic DNA
atgaaagtcgcagtcctcggcgctgctggcggtgtcggccaggcgcttgcactactgttaaaaacccaactgccttcaggttcagaactctctctgtatgatatcgctccagtgactcccggtgtggctgtcgatctgagccatatccctactgctgtgaaaatcaaaggtttttctggtgaagatgcgactccggcgctggaaggcgcagatgtcgttcttatctctgcaggcgtagcggctaaacccgggatggatcgttccgacctgtttaacgttaacgccggcatcgtgaaaaacctggtacagcaagttgcgaaaacctgcccgaaagcgtgcattggtattatcactaacccggttaacaccacagttgcaattgctgctgaagtgctgaaaaaagccggtgtttatgacaaaaacaaactgttcggcgttaccacgctggatatcattcgttccaacacctttgttgcggaactgaaaggcaaacagccaggcgaagttgaagtgccggttattggcggtcactctggtgttaccattctgccgctgctgtcacaggttcctggcgttagttttaccgagcaggaagtggctgatctgaccaaacgcatccagaacgcgggtactgaagtggttgaagcgaaggccggtggcgggtctgcaaccctgtctatgggccaggcagctgcacgttttggtctgtctctggttcgtgcactgcagggcgaacaaggcgttgtcgaatgtgcctacgttgaaggcgacggtcagtacgcccgtttcttctctcaaccgctgctgctgggtaaaaacggcgtggaagagcgtaaatctatcggtaccctgagcgcatttgaacagaacgcgctggaaggtatgctggatacgctgaagaaagatatcgccctgggcgaagagttcgttaataagtaa

SEQ ID NO: 80 - protein, 312 aa, Escherichia coli; identical to SEQ ID NO: 42

SEQ ID NO: 81 - DNA, 939 bp, Escherichia coli
  source 1..939: mol_type = genomic DNA
atgaaagtcgcagtcctcggcgctgctggcggtattggccaggcgcttgcactactgttaaaaacccaactgccttcaggttcagaactctctctgtatgatatcgctccagtgactcccggtgtggctgtcgatctgagccatatccctactgctgtgaaaatcaaaggtttttctggtgaagatgcgactccggcgctggaaggcgcagatgtcgttcttatctctgcaggcgtagcggctaaacccgggatgtctcgttccgacctgtttaacgttaacgccggcatcgtgaaaaacctggtacagcaagttgcgaaaacctgcccgaaagcgtgcattggtattatcactaacccggttaacaccacagttgcaattgctgctgaagtgctgaaaaaagccggtgtttatgacaaaaacaaactgttcggcgttaccacgctggatatcattcgttccaacacctttgttgcggaactgaaaggcaaacagccaggcgaagttgaagtgccggttattggcggccactctgatgttaccattctgccgctgctgtcacaggttcctggcgttagttttaccgagcaggaagtggctgatctgaccaaacgcatccagaacgcgggtactgaagtggttgaagcgaaggccggtggcgggtctgcaaccctgtctatgggccaggcagctgcacgttttggtctgtctctggttcgtgcactgcagggcgaacaaggcgttgtcgaatgtgcctacgttgaaggcgacggtcagtacgcccgtttcttctctcaaccgctgctgctgggtaaaaacggcgtggaagagcgtaaatctatcggtaccctgagcgcatttgaacagaacgcgctggaaggtatgctggatacgctgaagaaagatatcgccctgggcgaagagttcgttaataagtaa

SEQ ID NO: 82 - protein, 312 aa, Escherichia coli; identical to SEQ ID NO: 44

SEQ ID NO: 83 - DNA, 19 bp, synthetic construct
  source 1..19: mol_type = other DNA
aggtcagcgaatttctctc

SEQ ID NO: 84 - DNA, 22 bp, synthetic construct
  source 1..22: mol_type = other DNA
gatacatcacttgccataagtc

SEQ ID NO: 85 - DNA, 20 bp, synthetic construct
  source 1..20: mol_type = other DNA
tcattcgtgtgaatggacag

SEQ ID NO: 86 - DNA, 19 bp, synthetic construct
  source 1..19: mol_type = other DNA
taagccggaaattgatggc

SEQ ID NO: 87 - DNA, 18 bp, synthetic construct
  source 1..18: mol_type = other DNA
cgccgaaagagattgttg

SEQ ID NO: 88 - DNA, 20 bp, synthetic construct
  source 1..20: mol_type = other DNA
agcaatcacgtcagcaatag

SEQ ID NO: 89 - DNA, 16 bp, synthetic construct
  source 1..16: mol_type = other DNA
cgccagtaaatctgcc

SEQ ID NO: 90 - DNA, 16 bp, synthetic construct
  source 1..16: mol_type = other DNA
aggcgggatgaagatg

SEQ ID NO: 91 - DNA, 20 bp, synthetic construct
  source 1..20: mol_type = other DNA
atgatatcgaagcctcaatc

SEQ ID NO: 92 - DNA, 20 bp, synthetic construct
  source 1..20: mol_type = other DNA
ttatcaggcctacaaattcc

SEQ ID NO: 93 - DNA, 60 bp, synthetic construct
  source 1..60: mol_type = other DNA
gtcctaggtataatactagtcggtaaaaaactttatatctgttttagagctagaaatagc

SEQ ID NO: 94 - DNA, 26 bp, synthetic construct
  source 1..26: mol_type = other DNA
gtcgttgatcaaagctcgccgcgttg

SEQ ID NO: 95 - DNA, 23 bp, synthetic construct
  source 1..23: mol_type = other DNA
gatctgcgcaacaacaaataatg

SEQ ID NO: 96 - DNA, 16 bp, synthetic construct
  source 1..16: mol_type = other DNA
catgccgcttctcctg

SEQ ID NO: 97 - DNA, 24 bp, synthetic construct
  source 1..24: mol_type = other DNA
actagtattatacctaggactgag

SEQ ID NO: 98 - DNA, 19 bp, synthetic construct
  source 1..19: mol_type = other DNA
gttattgtctcatgagcgg

SEQ ID NO: 99 - DNA, 19 bp, synthetic construct
  source 1..19: mol_type = other DNA
ctttgagtgagctgatacc

SEQ ID NO: 100 - DNA, 20 bp, synthetic construct
  source 1..20: mol_type = other DNA
ccgaacaagtgttcactatg

SEQ ID NO: 101 - DNA, 20 bp, synthetic construct
  source 1..20: mol_type = other DNA
gataatcagcacctctttgc

SEQ ID NO: 102 - DNA, 20 bp, synthetic construct
  source 1..20: mol_type = other DNA
tgcagctatcgggtttattg

SEQ ID NO: 103 - DNA, 20 bp, synthetic construct
  source 1..20: mol_type = other DNA
tgctgatattccgaactgtc

SEQ ID NO: 104 - DNA, 20 bp, synthetic construct
  source 1..20: mol_type = other DNA
agaattacaaaaaacacgcc

SEQ ID NO: 105 - DNA, 20 bp, synthetic construct
  source 1..20: mol_type = other DNA
ctgagcagtaaaataccgtc

SEQ ID NO: 106 - DNA, 21 bp, synthetic construct
  source 1..21: mol_type = other DNA
catgctagccatatggctgcc

SEQ ID NO: 107 - DNA, 22 bp, synthetic construct
  source 1..22: mol_type = other DNA
atgcctcgagcaccaccaccac

SEQ ID NO: 108 - DNA, 31 bp, synthetic construct
  source 1..31: mol_type = other DNA
tcacatatgatgaaaaactggaaaacaagtg

SEQ ID NO: 109 - DNA, 31 bp, synthetic construct
  source 1..31: mol_type = other DNA
tgacctcgagttacagcttagcgccttctac

SEQ ID NO: 110 - DNA, 27 bp, synthetic construct
  source 1..27: mol_type = other DNA
gatcaggatccatgaacggtaaaaaac

SEQ ID NO: 111 - DNA, 27 bp, synthetic construct
  source 1..27: mol_type = other DNA
cagtcaagcttttatttgttgttgcgc

SEQ ID NO: 112 - DNA, 27 bp, synthetic construct
  source 1..27: mol_type = other DNA
tcacctagggccgctgctgtgatgatg

SEQ ID NO: 113 - DNA, 28 bp, synthetic construct
  source 1..28: mol_type = other DNA
atccaattgtgagatccggctgctaaca

SEQ ID NO: 114 - DNA, 28 bp, synthetic construct
  source 1..28: mol_type = other DNA
atccctaggatgcagtggcaaactaaac

SEQ ID NO: 115 - DNA, 26 bp, synthetic construct
  source 1..26: mol_type = other DNA
atccaattgtcattgcactgcctctc

SEQ ID NO: 116 - DNA, 30 bp, synthetic construct
  source 1..30: mol_type = other DNA
atccctaggatgaataacgatgttttcccg

SEQ ID NO: 117 - DNA, 33 bp, synthetic construct
  source 1..33: mol_type = other DNA
atccaattgttattttttaaaggtatcagccag

SEQ ID NO: 118 - DNA, 25 bp, synthetic construct
  source 1..25: mol_type = other DNA
atccctaggatgccgcagtccgcgt

SEQ ID NO: 119 - DNA, 31 bp, synthetic construct
  source 1..31: mol_type = other DNA
tcacaattgtcagcaaagcttgagctgttgc

SEQ ID NO: 120 - DNA, 31 bp, synthetic construct
  source 1..31: mol_type = other DNA
tcacctaggatgaacgcattattaagcaatc

SEQ ID NO: 121 - DNA, 30 bp, synthetic construct
  source 1..30: mol_type = other DNA
tcacattgtcaataactaccttttatgcgt

SEQ ID NO: 122 - DNA, 27 bp, synthetic construct
  source 1..27: mol_type = other DNA
tcacctaggatgaaaaaattcagcggc

SEQ ID NO: 123 - DNA, 28 bp, synthetic construct
  source 1..28: mol_type = other DNA
tcacaattgtcagactggtaaaatgccc

SEQ ID NO: 124 - DNA, 15 bp, synthetic construct
  source 1..15: mol_type = other DNA
cgagatctcgatccc

SEQ ID NO: 125 - DNA, 18 bp, synthetic construct
  source 1..18: mol_type = other DNA
tccggatatagttcctcc

SEQ ID NO: 126 - DNA, 1239 bp, Escherichia coli
  source 1..1239: mol_type = genomic DNA
atggctgacactcgccctgaacgtcgctttacgcgcattgatcgtctcccgccctacgtttttaacatcaccgctgaactgaaaatggctgcgcgtcggcgcggcgaagatattatcgatttcagcatgggtaacccggacggtgcgactccgccgcatatcgtcgaaaaattatgtactgtggcccagcgcccggacacgcatggttactccacttcacgcggcattccgcggttacgtcgcgccatttcccgctggtatcaggatcgctacgacgttgaaatcgacccggaatcagaagccatcgtcactattggttcgaaagagggcctggcgcatctgatgctggcgacgctggatcatggtgacacggtgctggtgccgaatccaagttacccgatccatatttatggcgcggtgattgccggggcgcaggtacgctcagtgccgctggtggaaggtgtcgatttcttcaacgaactggagcgagccattcgtgaaagttatccgaaaccgaagatgatgatcctcggcttcccgtcaaacccaaccgcgcaatgcgtggaactggagttcttcgaaaaagtagtggcgctggcgaaacgctacgatgtgctggtggtccatgacctggcctatgccgatatcgtctacgatggctggaaagcgccgtcaattatgcaggtaccgggtgcacgcgatgtggcagtcgagttctttacgctgtcgaaaagctacaacatggcgggctggcgtatcggctttatggttggcaacaaaacgctggtcagcgccctggctcgtattaaaagctatcacgattacggcacctttacgccgttgcaggtggcggcgattgcggcgctggagggcgatcaacagtgcgtgcgcgacattgccgaacagtacaaacgccgccgtgatgtattggttaaagggctgcatgaagcgggctggatggttgaaatgccgaaggcttcgatgtatgtctgggcgaaaatcccggaaccatatgcggccatgggatcgctggaatttgccaagaagctccttaacgaagcgaaggtttgtgtctcgccggggattggctttggcgactatggtgatacgcatgttcgctttgcactgattgaaaaccgcgaccgtattcgtcaggccatcagagggattaaagcgatgttccgtgccgacggtttactacccgccagcagcaaacatattcacgaaaacgcggaataa

SEQ ID NO: 127 - protein, 412 aa, Escherichia coli
MADTRPERRFTRIDRLPPYVFNITAELKMAARRRGEDIIDFSMGNPDGATPPHIVEKLCTVAQRPDTHGYSTSRGIPRLRRAISRWYQDRYDVEIDPESEAIVTIGSKEGLAHLMLATLDHGDTVLVPNPSYPIHIYGAVIAGAQVRSVPLVEGVDFFNELERAIRESYPKPKMMILGFPSNPTAQCVELEFFEKVVALAKRYDVLVVHDLAYADIVYDGWKAPSIMQVPGARDVAVEFFTLSKSYNMAGWRIGFMVGNKTLVSALARIKSYHDYGTFTPLQVAAIAALEGDQQCVRDIAEQYKRRRDVLVKGLHEAGWMVEMPKASMYVWAKIPEPYAAMGSLEFAKKLLNEAKVCVSPGIGFGDYGDTHVRFALIENRDRIRQAIRGIKAMFRADGLLPASSKHIHENAE

SEQ ID NO: 128 - DNA, 1239 bp, Escherichia coli
  source 1..1239: mol_type = genomic DNA
atggctgacactcgccctgaacgtcgctttacgcgcattgatcgtctcccgccctacgtttttaacatcaccgctgaactgaaaatggctgcgcgtcggcgcggcgaagatattatcgatttcagcatgggtaacccggacggtgcgactccgccgcatatcgtcgaaaaattatgtactgtggcccagcgcccggacacgcatggttactccacttcacgcggcattccgcggttacgtcgcgccatttcccgctggtatcaggatcgctacgacgttgaaatcgacccggaatcagaagccatcgtcactattggttcgaaagagggcctggcgcatctgatgctggcgacgctggatcatggtgacacggtgctggtgccgaatccaagttacccgatccatatttatggcgcggtgattcccggggcgcaggtacgctcagtgccgctggtggaaggtgtcgatttcttcaacgaactggagcgagccattcgtgaaagttatccgaaaccgaagatgatgatcctcggcttcccgtcaaacccaaccgcgcaatgcgtggaactggagttcttcgaaaaagtagtggcgctggcgaaacgctacgatgtgctggtggtccatgacctggcctatgccgatatcgtctacgatggctggaaagcgccgtcaattatgcaggtaccgggtgcacgcgatgtggcagtcgagttctttacgctgtcgaaaagctacaacatggcgggctggcgtatcggctttatggttggcaacaaaacgctggtcagcgccctggctcgtattaaaagctatcacgatgacggcacctttacgccgttgcaggtggcggcgattgcggcgctggagggcgatcaacagtgcgtgcgcgacattgccgaacagtacaaacgccgccgtgatgtattggttaaagggctgcatgaagcgggctggatggttgaaatgccgaaggcttcgatgtatgtctgggcgaaaatcccggaaccatatgcggccatgggatcgctggaatttgccaagaagctccttaacgaagcgaaggtttgtgtctcgccggggattggctttggcgactatggtgatacgcatgttcgctttgcactgattgaaaaccgcgaccgtattcgtcaggccatcagagggattaaagcgatgttccgtgccgacggtttactacccgccagcagcaaacatattcacgaaaacgcggaataa

SEQ ID NO: 129 - protein, 412 aa, Escherichia coli
MADTRPERRFTRIDRLPPYVFNITAELKMAARRRGEDIIDFSMGNPDGATPPHIVEKLCTVAQRPDTHGYSTSRGIPRLRRAISRWYQDRYDVEIDPESEAIVTIGSKEGLAHLMLATLDHGDTVLVPNPSYPIHIYGAVIPGAQVRSVPLVEGVDFFNELERAIRESYPKPKMMILGFPSNPTAQCVELEFFEKVVALAKRYDVLVVHDLAYADIVYDGWKAPSIMQVPGARDVAVEFFTLSKSYNMAGWRIGFMVGNKTLVSALARIKSYHDDGTFTPLQVAAIAALEGDQQCVRDIAEQYKRRRDVLVKGLHEAGWMVEMPKASMYVWAKIPEPYAAMGSLEFAKKLLNEAKVCVSPGIGFGDYGDTHVRFALIENRDRIRQAIRGIKAMFRADGLLPASSKHIHENAE

SEQ ID NO: 130 - DNA, 19 bp, synthetic construct
  source 1..19: mol_type = other DNA
tgtgcttaacccagcagag

SEQ ID NO: 131 - DNA, 18 bp, synthetic construct
  source 1..18: mol_type = other DNA
tacgggcgaaatgtaggc